European Patent Application EP 4 186 926 A1, published May 31, 2023. Title: CCR8 ANTIBODY AND APPLICATION THEREOF. Applicant: Harbour BioMed US, Inc. Application EP 21 860 522.8. The sequence listing filed with the application follows.

SEQUENCE LISTING (368 sequences)

SEQ ID NO: 1 - protein, 25 aa, Artificial Sequence
  H-FR1
EVQLVESGGGLVQPKGSLKLSCAAS

SEQ ID NO: 2 - protein, 25 aa, Artificial Sequence
  PR004122|pHBM005089-VH|H-FR1; PR004127|pHBM005094-VH|H-FR1; PR004249|pHBM005373-VH|H-FR1
EVQLVETGGGLVQPKGSLKLSCAAS

SEQ ID NO: 3 - protein, 25 aa, Artificial Sequence
  PR004124|pHBM005091-VH|H-FR1
EVKVEESGGGLVQPGGSMKLSCAAS

SEQ ID NO: 4 - protein, 25 aa, Artificial Sequence
  PR004130|pHBM005096-VH|H-FR1
EVQLVESGGGLVQFKGSLKLSCGTS

SEQ ID NO: 5 - protein, 25 aa, Artificial Sequence [sequence omitted]

SEQ ID NO: 6 - protein, 25 aa, Artificial Sequence
  PR004265|pHBM005403-VH|H-FR1
EVQLVESGGGLVQPGGSRKLSCAAS

SEQ ID NO: 7 - protein, 25 aa, Artificial Sequence
  H-FR1
EVQLVESGGGLVKPGGSLRLSCAAS

SEQ ID NO: 8 - protein, 25 aa, Artificial Sequence
  H-FR1
EVQLVESGGGLVQPGGSLKLSCAAS

SEQ ID NO: 9 - protein, 25 aa, Artificial Sequence
  PR004974|pHBM006117-VH|H-FR1; PR005293|pHBM006504-VH|H-FR1
QITLKESGPTLVKPTQTLTLTCTFS

SEQ ID NO: 10 - protein, 25 aa, Artificial Sequence
  PR005124|pHBM006274-VH|H-FR1; PR005127|pHBM006280-VH|H-FR1
QVQLVESGGGVVQPGRSLRLSCVAS

SEQ ID NO: 11 - protein, 25 aa, Artificial Sequence
  PR005125|pHBM006276-VH|H-FR1; PR005128|pHBM006281-VH|H-FR1
QVQLVESGGGVVQPGRSLRLSCAAS

SEQ ID NO: 12 - protein, 25 aa, Artificial Sequence
  PR005329|pHBM006537-VH|H-FR1; PR005332|pHBM006540-VH|H-FR1
EVKLLESGGGLVQPKGSLKLSCAAS

SEQ ID NO: 13 - protein, 25 aa, Artificial Sequence
  PR005330|pHBM006538-VH|H-FR1; PR005333|pHBM006541-VH|H-FR1
EVKLVESGGGLVQPGGSRKLSCAAS

SEQ ID NO: 14 - protein, 25 aa, Artificial Sequence
  PR005335|pHBM006543-VH|H-FR1
QVQLVQSGGGLVQPGGSLRLSCTAS

SEQ ID NO: 15 - protein, 7 aa, Artificial Sequence
  HCDR1
GFTFNTN

SEQ ID NO: 16 - protein, 7 aa, Artificial Sequence
  HCDR1
GFTFNTY

SEQ ID NO: 17 - protein, 7 aa, Artificial Sequence
  PR004123|pHBM005090-VH|HCDR1
EFTFNTY

SEQ ID NO: 18 - protein, 7 aa, Artificial Sequence
  PR004126|pHBM005093-VH|HCDR1
GFTFSTN

SEQ ID NO: 19 - protein, 7 aa, Artificial Sequence
  HCDR1
GFTFSSY

SEQ ID NO: 20 - protein, 7 aa, Artificial Sequence
  PR004265|pHBM005403-VH|HCDR1
GFTFSSF

SEQ ID NO: 21 - protein, 7 aa, Artificial Sequence
  PR004327|pHBM005431-VH|HCDR1
GFTFQTY

SEQ ID NO: 22 - protein, 7 aa, Artificial Sequence
  HCDR1
GFTFSTY

SEQ ID NO: 23 - protein, 9 aa, Artificial Sequence
  PR004974|pHBM006117-VH|HCDR1; PR005293|pHBM006504-VH|HCDR1
GFSLSTSGV

SEQ ID NO: 24 - protein, 7 aa, Artificial Sequence
  PR005331|pHBM006539-VH|HCDR1; PR005336|pHBM006544-VH|HCDR1
GFTFSNY

SEQ ID NO: 25 - protein, 7 aa, Artificial Sequence
  PR005335|pHBM006543-VH|HCDR1
GFTFSYY

SEQ ID NO: 26 - protein, 19 aa, Artificial Sequence
  H-FR2
AMNWVRQAPGKGLEWVARI

SEQ ID NO: 27 - protein, 19 aa, Artificial Sequence
  H-FR2
AMNWVRQAPGKGLEWVGRI

SEQ ID NO: 28 - protein, 19 aa, Artificial Sequence
  PR004264|pHBM005401-VH|H-FR2; PR004275|pHBM005295-VH|H-FR2
AMSWVRQAPGKGLEWVSAI

SEQ ID NO: 29 - protein, 19 aa, Artificial Sequence
  PR004265|pHBM005403-VH|H-FR2
GMHWVRQVPEKGLEWVAYI

SEQ ID NO: 30 - protein, 19 aa, Artificial Sequence
  H-FR2
AMNWVRQAPGKGLEWVSRI

SEQ ID NO: 31 - protein, 19 aa, Artificial Sequence
  H-FR2
AMNWVRQASGKGLEWVGRI

SEQ ID NO: 32 - protein, 19 aa, Artificial Sequence
  PR004970|pHBM006115-VH|H-FR2
WMSWVPQAPGKGLEWVANI

SEQ ID NO: 33 - protein, 19 aa, Artificial Sequence
  PR004974|pHBM006117-VH|H-FR2; PR005293|pHBM006504-VH|H-FR2
GVGWIRQPPGKALEWLALI

SEQ ID NO: 34 - protein, 19 aa, Artificial Sequence
  PR005124|pHBM006274-VH|H-FR2; PR005127|pHBM006280-VH|H-FR2
GMHWVRQAPGKGLEWVAVI

SEQ ID NO: 35 - protein, 19 aa, Artificial Sequence
  PR005125|pHBM006276-VH|H-FR2; PR005128|pHBM006281-VH|H-FR2
GMHWVRQVPGKGLEWVAVI

SEQ ID NO: 36 - protein, 19 aa, Artificial Sequence
  PR005331|pHBM006539-VH|H-FR2; PR005335|pHBM006543-VH|H-FR2; PR005336|pHBM006544-VH|H-FR2
WLSWVRQAPGKGLEWVANI

SEQ ID NO: 37 - protein, 8 aa, Artificial Sequence
  PR004120|pHBM005087-VH|HCDR2
RSKMNNYA

SEQ ID NO: 38 - protein, 8 aa, Artificial Sequence
  HCDR2
RSKSNNYA

SEQ ID NO: 39 - protein, 8 aa, Artificial Sequence
  PR004123|pHBM005090-VH|HCDR2
RTKSNNFA

SEQ ID NO: 40 - protein, 6 aa, Artificial Sequence
  PR004264|pHBM005401-VH|HCDR2; PR004275|pHBM005295-VH|HCDR2
SGSGGS

SEQ ID NO: 41 - protein, 6 aa, Artificial Sequence
  PR004265|pHBM005403-VH|HCDR2
SSGSRT

SEQ ID NO: 42 - protein, 6 aa, Artificial Sequence
  PR004970|pHBM006115-VH|HCDR2; PR005331|pHBM006539-VH|HCDR2; PR005336|pHBM006544-VH|HCDR2
KQDGSA

SEQ ID NO: 43 - protein, 5 aa, Artificial Sequence
  PR004974|pHBM006117-VH|HCDR2; PR005293|pHBM006504-VH|HCDR2
YWNDD

SEQ ID NO: 44 - protein, 6 aa, Artificial Sequence
  PR005124|pHBM006274-VH|HCDR2; PR005127|pHBM006280-VH|HCDR2
WHDGSN

SEQ ID NO: 45 - protein, 6 aa, Artificial Sequence
  PR005125|pHBM006276-VH|HCDR2; PR005128|pHBM006281-VH|HCDR2
WYDGSK

SEQ ID NO: 46 - protein, 8 aa, Artificial Sequence
  PR005329|pHBM006537-VH|HCDR2; PR005332|pHBM006540-VH|HCDR2
RTKSNNYA

SEQ ID NO: 47 - protein, 6 aa, Artificial Sequence
  PR005335|pHBM006543-VH|HCDR2
KQDGST

SEQ ID NO: 48 - protein, 8 aa, Artificial Sequence
  HCDR2
RSKSNYYA

SEQ ID NO: 49 - protein, 41 aa, Artificial Sequence
  PR004120|pHBM005087-VH|H-FR3; PR004121|pHBM005088-VH|H-FR3; PR004127|pHBM005094-VH|H-FR3
TYYADSVKDRFTISRDDSQNMLYLQMNNLKTEDTAMYYCVR

SEQ ID NO: 50 - protein, 41 aa, Artificial Sequence
  H-FR3
TYYADSVKDRFTISRDDSQSMLYLQMNNLKTEDTAMYYCVR

SEQ ID NO: 51 - protein, 41 aa, Artificial Sequence
  PR004123|pHBM005090-VH|H-FR3
TYYADSVKDRFTISRDDSQSMLFLQMNNLKTEDTAMYYCVR

SEQ ID NO: 52 - protein, 41 aa, Artificial Sequence
  PR004130|pHBM005096-VH|H-FR3
TFYADSVKDRFTISRDDSQNMLYLQMNNLKTEDTAMYYCVR

SEQ ID NO: 53 - protein, 41 aa, Artificial Sequence
  PR004264|pHBM005401-VH|H-FR3
TYYADSVKGRFTISRDNSKNTLYLQMNSLRAEDTAVYYCAT

SEQ ID NO: 54 - protein, 41 aa, Artificial Sequence
  PR004265|pHBM005403-VH|H-FR3
IYYTDTVKGRFTISRDNPKNTLFLQMTSLRSEDTAIYYCVR

SEQ ID NO: 55 - protein, 41 aa, Artificial Sequence
  PR004275|pHBM005295-VH|H-FR3
TYYADSVKGRFTISRDNSKNTLYLQMNSLRAEDTAVYYCAR

SEQ ID NO: 56 - protein, 41 aa, Artificial Sequence
  H-FR3
TYYADSVKDRFTISRDDSKSTLYLQMNSLKTEDTAVYYCVR

SEQ ID NO: 57 - protein, 41 aa, Artificial Sequence
  H-FR3
TYYADSVKDRFTISRDDSKSTLYLQMNSLRAEDTAVYYCVR

SEQ ID NO: 58 - protein, 41 aa, Artificial Sequence
  PR004970|pHBM006115-VH|H-FR3
KFYVDSVKGRFTISRDNAKNSLYLQMNSLRAEDTAVYYCAR

SEQ ID NO: 59 - protein, 41 aa, Artificial Sequence
  PR004974|pHBM006117-VH|H-FR3; PR005293|pHBM006504-VH|H-FR3
KRYSPSLKSRLTITKDTSKNQVVLTMTNMDPVDTATYYCAH

SEQ ID NO: 60 - protein, 41 aa, Artificial Sequence
  PR005124|pHBM006274-VH|H-FR3; PR005127|pHBM006280-VH|H-FR3
IFYADSVKGRFTISRDNSKNTLYLQMNSLRAEDTAVYWCAR

SEQ ID NO: 61 - protein, 41 aa, Artificial Sequence
  PR005125|pHBM006276-VH|H-FR3; PR005128|pHBM006281-VH|H-FR3
KYYADSVKGRFTISRDNSKNTLYLQMNSLRAEDTAVYYCAR

SEQ ID NO: 62 - protein, 41 aa, Artificial Sequence
  PR005329|pHBM006537-VH|H-FR3; PR005332|pHBM006540-VH|H-FR3
TYYADSVKDRFTISRDDSHSMLYLQMNNLKTEDTAMYYCVR

SEQ ID NO: 63 - protein, 41 aa, Artificial Sequence
  PR005331|pHBM006539-VH|H-FR3; PR005336|pHBM006544-VH|H-FR3
KYYVDSVKGRFTISRDNAKNSLYLQMNSLRAEDTAVYYCVR

SEQ ID NO: 64 - protein, 41 aa, Artificial Sequence
  PR005335|pHBM006543-VH|H-FR3
TYYVDSVKGRFTISRDNAKNSLYLQMNSLRAEDTAVYYCAR

SEQ ID NO: 65 - protein, 12 aa, Artificial Sequence
  HCDR3
GKENGNYYAMDF

SEQ ID NO: 66 - protein, 12 aa, Artificial Sequence
  PR004124|pHBM005091-VH|HCDR3; PR005330|pHBM006538-VH|HCDR3; PR005333|pHBM006541-VH|HCDR3
GKDYGNYYAMDF

SEQ ID NO: 67 - protein, 12 aa, Artificial Sequence
  PR004129|pHBM005095-VH|HCDR3
GKDYGNYYAMDY

SEQ ID NO: 68 - protein, 12 aa, Artificial Sequence
  HCDR3
GKENGNYYAMDY

SEQ ID NO: 69 - protein, 5 aa, Artificial Sequence
  PR004264|pHBM005401-VH|HCDR3
QGFDY

SEQ ID NO: 70 - protein, 11 aa, Artificial Sequence
  PR004265|pHBM005403-VH|HCDR3
GGLRPYWYFDV

SEQ ID NO: 71 - protein, 10 aa, Artificial Sequence
  PR004275|pHBM005295-VH|HCDR3
RWGKGGLFDY

SEQ ID NO: 72 - protein, 12 aa, Artificial Sequence
  HCDR3
GKENANYYAMDF

SEQ ID NO: 73 - protein, 12 aa, Artificial Sequence
  HCDR3
GKEQGNYYAMDF

SEQ ID NO: 74 - protein, 6 aa, Artificial Sequence
  PR004970|pHBM006115-VH|HCDR3
SWGFAY

SEQ ID NO: 75 - protein, 17 aa, Artificial Sequence
  PR004974|pHBM006117-VH|HCDR3; PR005293|pHBM006504-VH|HCDR3
RRLRYSGRYYYYYGTDV

SEQ ID NO: 76 - protein, 13 aa, Artificial Sequence
  PR005124|pHBM006274-VH|HCDR3; PR005127|pHBM006280-VH|HCDR3
HRRSDYWYYGMDV

SEQ ID NO: 77 - protein, 15 aa, Artificial Sequence
  PR005125|pHBM006276-VH|HCDR3; PR005128|pHBM006281-VH|HCDR3
GGFYYGSGNYSLFDY

SEQ ID NO: 78 - protein, 12 aa, Artificial Sequence
  PR005329|pHBM006537-VH|HCDR3; PR005332|pHBM006540-VH|HCDR3
GKDNGNYYAMDF

SEQ ID NO: 79 - protein, 6 aa, Artificial Sequence
  PR005331|pHBM006539-VH|HCDR3; PR005335|pHBM006543-VH|HCDR3; PR005336|pHBM006544-VH|HCDR3
NWGFDY

SEQ ID NO: 80 - protein, 12 aa, Artificial Sequence
  HCDR3
GKEHGNYYAMDF

SEQ ID NO: 81 - protein, 12 aa, Artificial Sequence
  HCDR3
GKEIGNYYAMDF

SEQ ID NO: 82 - protein, 12 aa, Artificial Sequence
  PR005763|pHBM007005-VH|HCDR3; PR006161|pHBM006987-VH|HCDR3; PR006274|pHBM007523-VH|HCDR3
GKEHGKYYAMDF

SEQ ID NO: 83 - protein, 12 aa, Artificial Sequence
  PR005787|pHBM007006-VH|HCDR3; PR006166|pHBM006988-VH|HCDR3; PR006275|pHBM007524-VH|HCDR3
GKEIGKYYAMDF

SEQ ID NO: 84 - protein, 11 aa, Artificial Sequence
  PR004120|pHBM005087-VH|H-FR4; PR004123|pHBM005090-VH|H-FR4; PR004125|pHBM005092-VH|H-FR4; PR004126|pHBM005093-VH|H-FR4; PR004128|pHBM005092-VH|H-FR4; PR004250|pHBM005374-VH|H-FR4; PR004251|pHBM005374-VH|H-FR4; PR004324|pHBM005374-VH|H-FR4; PR004325|pHBM005374-VH|H-FR4; PR004326|pHBM005430-VH|H-FR4; PR004327|pHBM005431-VH|H-FR4; PR004328|pHBM005432-VH|H-FR4; PR004329|pHBM005433-VH|H-FR4; PR004339|pHBM005374-VH|H-FR4; PR004340|pHBM005374-VH|H-FR4; PR004342|pHBM005374-VH|H-FR4; PR004343|pHBM005374-VH|H-FR4; PR004344|pHBM005374-VH|H-FR4; PR004345|pHBM005374-VH|H-FR4; PR004346|pHBM005374-VH|H-FR4; PR005170|pHBM005092-VH|H-FR4; PR005171|pHBM005092-VH|H-FR4; PR005172|pHBM005092-VH|H-FR4; PR005329|pHBM006537-VH|H-FR4; PR005332|pHBM006540-VH|H-FR4
WGQGTSVTVSA

SEQ ID NO: 85 - protein, 11 aa, Artificial Sequence
  |H-FR4
WGQGTSVTVSS

SEQ ID NO: 86 - protein, 11 aa, Artificial Sequence
  PR004124|pHBM005091-VH|H-FR4
WGQGTSLTVSS

SEQ ID NO: 87 - protein, 11 aa, Artificial Sequence
  H-FR4
WGQGTLVTVSS

SEQ ID NO: 88 - protein, 11 aa, Artificial Sequence
  PR004265|pHBM005403-VH|H-FR4
WGAGTTVTVSA

SEQ ID NO: 89 - protein, 11 aa, Artificial Sequence
  H-FR4
WGQGTTVTVSS

SEQ ID NO: 90 - protein, 23 aa, Artificial Sequence
  L-FR1
DIVMTQAATSVLVTPGESVSISC

SEQ ID NO: 91 - protein, 23 aa, Artificial Sequence
  PR004121|pHBM005099-VL|L-FR1; PR004126|pHBM005104-VL|L-FR1
DIVITQAAPSVPVTPGESVSISC

SEQ ID NO: 92 - protein, 23 aa, Artificial Sequence
  |L-FR1
DIVMTQAAPSVPVTPGESVSISC

SEQ ID NO: 93 - protein, 23 aa, Artificial Sequence
  PR004124|pHBM005102-VL|L-FR1
DIVMTQDELSNPVTSGESVSISC

SEQ ID NO: 94 - protein, 23 aa, Artificial Sequence
  PR004129|pHBM005107-VL|L-FR1
DILLTQSPAILSVSPGERVSFSC

SEQ ID NO: 95 - protein, 23 aa, Artificial Sequence
  PR004264|pHBM005402-VL|L-FR1; PR005335|pHBM006548-VL|L-FR1
DVVMTQSPLSLPVTLGQPASISC

SEQ ID NO: 96 - protein, 23 aa, Artificial Sequence
  PR004265|pHBM005404-VL|L-FR1
DIVLIQSPAIMSASPGEKVTISC

SEQ ID NO: 97 - protein, 23 aa, Artificial Sequence
  PR004275|pHBM005296-VL|L-FR1
DIQLTQSPSTLSASVGDRVTITC

SEQ ID NO: 98 - protein, 23 aa, Artificial Sequence
  L-FR1
DIVMTQSPLSLPVTPGEPASISC

SEQ ID NO: 99 - protein, 23 aa, Artificial Sequence
  L-FR1
DIVMTQSPLSLPVTLGQPASISC

SEQ ID NO: 100 - protein, 23 aa, Artificial Sequence
  PR004970|pHBM006122-VL|L-FR1
DIQMTQSPSSLSASVGDRVTITC

SEQ ID NO: 101 - protein, 23 aa, Artificial Sequence
  PR004974|pHBM006126-VL|L-FR1; PR005293|pHBM006126-VL|L-FR1
EIVMTQSPATLSVSPGERATLSC

SEQ ID NO: 102 - protein, 23 aa, Artificial Sequence
  PR005124|pHBM006275-VL|L-FR1; PR005127|pHBM006275-VL|L-FR1
DVVMTQSPLSLPVTPGEPASISC

SEQ ID NO: 103 - protein, 23 aa, Artificial Sequence
  PR005125|pHBM006277-VL|L-FR1; PR005128|pHBM006277-VL|L-FR1
DIVMTQSPLSLSVTLGQPASISC

SEQ ID NO: 104 - protein, 16 aa, Artificial Sequence
  PR004120|pHBM005098-VL|LCDR1; PR004127|pHBM005105-VL|LCDR1; PR005330|pHBM006546-VL|LCDR1; PR005333|pHBM006546-VL|LCDR1
RSSKSLLYSNGNTYLY

SEQ ID NO: 105 - protein, 16 aa, Artificial Sequence
  PR004121|pHBM005099-VL|LCDR1; PR004122|pHBM005100-VL|LCDR1; PR004123|pHBM005101-VL|LCDR1; PR004124|pHBM005102-VL|LCDR1
RSSKSLLHSNGNTYLY

SEQ ID NO: 106 - protein, 16 aa, Artificial Sequence
  LCDR1
RSSKSLLHSNGKIYLY

SEQ ID NO: 107 - protein, 16 aa, Artificial Sequence
  PR004131|pHBM005109-VL|LCDR1; PR004252|pHBM005109-VL|LCDR1; PR004345|pHBM005454-VL|LCDR1
RSNKSLLHSNGNTYLY

SEQ ID NO: 108 - protein, 16 aa, Artificial Sequence
  PR004264|pHBM005402-VL|LCDR1
RSSQSLVYSDGNTYLN

SEQ ID NO: 109 - protein, 10 aa, Artificial Sequence
  PR004265|pHBM005404-VL|LCDR1
SASSSVSYMY

SEQ ID NO: 110 - protein, 11 aa, Artificial Sequence
  PR004275|pHBM005296-VL|LCDR1
RASQSISSWLA

SEQ ID NO: 111 - protein, 16 aa, Artificial Sequence
  PR004324|pHBM005456-VL|LCDR1; PR004662|pHBM005790-VL|LCDR1
RSSKSLLHSNAKIYLY

SEQ ID NO: 112 - protein, 16 aa, Artificial Sequence
  PR004325|pHBM005457-VL|LCDR1
RSSKSLLHSQGKIYLY

SEQ ID NO: 113 - protein, 11 aa, Artificial Sequence
  PR004970|pHBM006122-VL|LCDR1
RASQGISNYLA

SEQ ID NO: 114 - protein, 11 aa, Artificial Sequence
  PR004974|pHBM006126-VL|LCDR1; PR005293|pHBM006126-VL|LCDR1
RASQSVSSNLV

SEQ ID NO: 115 - protein, 16 aa, Artificial Sequence
  PR005124|pHBM006275-VL|LCDR1; PR005127|pHBM006275-VL|LCDR1
RSSQSLLHSNGYNYLD

SEQ ID NO: 116 - protein, 16 aa, Artificial Sequence
  PR005125|pHBM006277-VL|LCDR1; PR005128|pHBM006277-VL|LCDR1
RSSQSLVFSNGNTYLN

SEQ ID NO: 117 - protein, 16 aa, Artificial Sequence
  PR005331|pHBM006549-VL|LCDR1; PR005335|pHBM006548-VL|LCDR1; PR005336|pHBM006549-VL|LCDR1
RSSQSLVYSNGNTYLN

SEQ ID NO: 118 - protein, 15 aa, Artificial Sequence
  L-FR2
WFLQRPGQSPQLLIY

SEQ ID NO: 119 - protein, 15 aa, Artificial Sequence
  PR004264|pHBM005402-VL|L-FR2; PR005125|pHBM006277-VL|L-FR2; PR005128|pHBM006277-VL|L-FR2; PR005331|pHBM006549-VL|L-FR2; PR005335|pHBM006548-VL|L-FR2; PR005336|pHBM006549-VL|L-FR2
WFQQRPGQSPRRLIY

SEQ ID NO: 120 - protein, 15 aa, Artificial Sequence
  PR004265|pHBM005404-VL|L-FR2
WYQQKPGSSPKPWIY

SEQ ID NO: 121 - protein, 15 aa, Artificial Sequence
  PR004275|pHBM005296-VL|L-FR2
WYQQKPGKAPKLLIY

SEQ ID NO: 122 - protein, 15 aa, Artificial Sequence
  PR004339|pHBM005447-VL|L-FR2; PR004340|pHBM005448-VL|L-FR2; PR004342|pHBM005450-VL|L-FR2; PR004519|pHBM005447-VL|L-FR2
WFLQKPGQSPQLLIY

SEQ ID NO: 123 - protein, 15 aa, Artificial Sequence
  PR004343|pHBM005452-VL|L-FR2; PR004344|pHBM005453-VL|L-FR2; PR004345|pHBM005454-VL|L-FR2
WFQQRPGQSPRLLIY

SEQ ID NO: 124 - protein, 15 aa, Artificial Sequence
  PR004970|pHBM006122-VL|L-FR2
WYQQKPGKVPKLLIY

SEQ ID NO: 125 - protein, 15 aa, Artificial Sequence
  PR004974|pHBM006126-VL|L-FR2; PR005293|pHBM006126-VL|L-FR2
WYQQKPGQAPRLLIY

SEQ ID NO: 126 - protein, 15 aa, Artificial Sequence
  PR005124|pHBM006275-VL|L-FR2; PR005127|pHBM006275-VL|L-FR2
WYLQKPGQSPQLLIY

SEQ ID NO: 127 - protein, 7 aa, Artificial Sequence
  LCDR2
RMSNLAS

SEQ ID NO: 128 - protein, 7 aa, Artificial Sequence
  PR004264|pHBM005402-VL|LCDR2; PR005331|pHBM006549-VL|LCDR2; PR005335|pHBM006548-VL|LCDR2; PR005336|pHBM006549-VL|LCDR2
KVSNRDS

SEQ ID NO: 129 - protein, 7 aa, Artificial Sequence
  PR004265|pHBM005404-VL|LCDR2
RTSNLAS

SEQ ID NO: 130 - protein, 7 aa, Artificial Sequence
  PR004275|pHBM005296-VL|LCDR2
KASSLES

SEQ ID NO: 131 - protein, 7 aa, Artificial Sequence
  PR004970|pHBM006122-VL|LCDR2
AASTLQS

SEQ ID NO: 132 - protein, 7 aa, Artificial Sequence
  PR004974|pHBM006126-VL|LCDR2; PR005293|pHBM006126-VL|LCDR2
GASIRAT

SEQ ID NO: 133 - protein, 7 aa, Artificial Sequence
  PR005124|pHBM006275-VL|LCDR2; PR005127|pHBM006275-VL|LCDR2
LGSNRAS

SEQ ID NO: 134 - protein, 7 aa, Artificial Sequence
  PR005125|pHBM006277-VL|LCDR2; PR005128|pHBM006277-VL|LCDR2
KVSKRDS

SEQ ID NO: 135 - protein, 32 aa, Artificial Sequence
  L-FR3
GVPDRFSGSGSGTAFTLRISRVEAEDVGVYYC

SEQ ID NO: 136 - protein, 32 aa, Artificial Sequence
  L-FR3
GVPDRFSGSGSGTDFTLKISRVEAEDVGVYYC

SEQ ID NO: 137 - protein, 32 aa, Artificial Sequence
  PR004265|pHBM005404-VL|L-FR3
GVPARFSGSGSGTSYSLTISRMEAEDAATYYC

SEQ ID NO: 138 - protein, 32 aa, Artificial Sequence
  PR004275|pHBM005296-VL|L-FR3; PR004970|pHBM006122-VL|L-FR3
GVPSRFSGSGSGTDFTLTISSLQPEDVATYYC

SEQ ID NO: 139 - protein, 32 aa, Artificial Sequence
  PR004974|pHBM006126-VL|L-FR3; PR005293|pHBM006126-VL|L-FR3
GIPARFSGSGSGTEFTLTISSLQSEDFAVYYC

SEQ ID NO: 140 - protein, 32 aa, Artificial Sequence
  PR005329|pHBM006545-VL|L-FR3; PR005332|pHBM006545-VL|L-FR3
GVPDRFSSSGSGTDFTLRISRVEAEDVGVYYC

SEQ ID NO: 141 - protein, 9 aa, Artificial Sequence
  PR004120|pHBM005098-VL|LCDR3; PR004121|pHBM005099-VL|LCDR3; PR004123|pHBM005101-VL|LCDR3; PR004124|pHBM005102-VL|LCDR3; PR004126|pHBM005104-VL|LCDR3; PR004127|pHBM005105-VL|LCDR3; PR004129|pHBM005107-VL|LCDR3; PR004130|pHBM005108-VL|LCDR3; PR004342|pHBM005450-VL|LCDR3; PR004346|pHBM005455-VL|LCDR3; PR005329|pHBM006545-VL|LCDR3; PR005330|pHBM006546-VL|LCDR3; PR005332|pHBM006545-VL|LCDR3; PR005333|pHBM006546-VL|LCDR3
MQHLEYPFT

SEQ ID NO: 142 - protein, 9 aa, Artificial Sequence
  LCDR3
MQHLEYPLT

SEQ ID NO: 143 - protein, 10 aa, Artificial Sequence
  PR004264|pHBM005402-VL|LCDR3
MQGTHWPPIT

SEQ ID NO: 144 - protein, 9 aa, Artificial Sequence
  PR004265|pHBM005404-VL|LCDR3
QQRSSYPPT

SEQ ID NO: 145 - protein, 9 aa, Artificial Sequence
  PR004275|pHBM005296-VL|LCDR3
QKYNSAPPT

SEQ ID NO: 146 - protein, 9 aa, Artificial Sequence
  PR004970|pHBM006122-VL|LCDR3
QKYNSAPWT

SEQ ID NO: 147 - protein, 9 aa, Artificial Sequence
  PR004974|pHBM006126-VL|LCDR3; PR005293|pHBM006126-VL|LCDR3
QQYNNWPYT

SEQ ID NO: 148 - protein, 9 aa, Artificial Sequence
  PR005124|pHBM006275-VL|LCDR3; PR005127|pHBM006275-VL|LCDR3
MQALQTPYT

SEQ ID NO: 149 - protein, 8 aa, Artificial Sequence
  PR005125|pHBM006277-VL|LCDR3; PR005128|pHBM006277-VL|LCDR3
MQGTHWIT

SEQ ID NO: 150 - protein, 9 aa, Artificial Sequence
  PR005170|pHBM006323-VL|LCDR3
MQHLEYPIT

SEQ ID NO: 151 - protein, 9 aa, Artificial Sequence
  PR005171|pHBM006324-VL|LCDR3
MQHLEYPMT

SEQ ID NO: 152 - protein, 9 aa, Artificial Sequence
  PR005172|pHBM006325-VL|LCDR3
MQHLEYPVT

SEQ ID NO: 153 - protein, 9 aa, Artificial Sequence
  PR005331|pHBM006549-VL|LCDR3; PR005335|pHBM006548-VL|LCDR3; PR005336|pHBM006549-VL|LCDR3
MQGTHWPIT

SEQ ID NO: 154 - protein, 10 aa, Artificial Sequence
  PR004120|pHBM005098-VL|L-FR4
FGGGTKLEIK

SEQ ID NO: 155 - protein, 10 aa, Artificial Sequence
  PR004121|pHBM005099-VL|L-FR4; PR004127|pHBM005105-VL|L-FR4
FGGGTKLEMK

SEQ ID NO: 156 - protein, 10 aa, Artificial Sequence
  PR004122|pHBM005100-VL|L-FR4; PR004126|pHBM005104-VL|L-FR4; PR004249|pHBM005100-VL|L-FR4; PR004265|pHBM005404-VL|L-FR4
FGAGTKLELK

SEQ ID NO: 157 - protein, 10 aa, Artificial Sequence
  PR004123|pHBM005101-VL|L-FR4; PR004124|pHBM005102-VL|L-FR4; PR005330|pHBM006546-VL|L-FR4; PR005333|pHBM006546-VL|L-FR4
FGGGTKLELK

SEQ ID NO: 158 - protein, 10 aa, Artificial Sequence
  PR004125|pHBM005103-VL|L-FR4; PR004250|pHBM005103-VL|L-FR4
FGAGTKLEMK

SEQ ID NO: 159 - protein, 10 aa, Artificial Sequence
  PR004128|pHBM005106-VL|L-FR4; PR004131|pHBM005109-VL|L-FR4; PR004251|pHBM005106-VL|L-FR4; PR004252|pHBM005109-VL|L-FR4; PR004324|pHBM005456-VL|L-FR4; PR004325|pHBM005457-VL|L-FR4; PR004326|pHBM005106-VL|L-FR4; PR004327|pHBM005106-VL|L-FR4; PR004328|pHBM005106-VL|L-FR4; PR004329|pHBM005106-VL|L-FR4; PR004330|pHBM005106-VL|L-FR4; PR004331|pHBM005106-VL|L-FR4; PR004332|pHBM005106-VL|L-FR4; PR004333|pHBM005106-VL|L-FR4; PR004334|pHBM005106-VL|L-FR4; PR004335|pHBM005106-VL|L-FR4; PR004336|pHBM005106-VL|L-FR4; PR004337|pHBM005106-VL|L-FR4; PR004338|pHBM005106-VL|L-FR4; PR005170|pHBM006323-VL|L-FR4; PR005171|pHBM006324-VL|L-FR4; PR005172|pHBM006325-VL|L-FR4; PR005329|pHBM006545-VL|L-FR4; PR005332|pHBM006545-VL|L-FR4
FGAGTKLEIK

SEQ ID NO: 160 - protein, 10 aa, Artificial Sequence
  PR004129|pHBM005107-VL|L-FR4
FGSGTKLEIN

SEQ ID NO: 161 - protein, 10 aa, Artificial Sequence
  PR004130|pHBM005108-VL|L-FR4
FGSGTKLEIK

SEQ ID NO: 162 - protein, 10 aa, Artificial Sequence
  PR004264|pHBM005402-VL|L-FR4; PR005125|pHBM006277-VL|L-FR4; PR005128|pHBM006277-VL|L-FR4; PR005331|pHBM006549-VL|L-FR4; PR005335|pHBM006548-VL|L-FR4; PR005336|pHBM006549-VL|L-FR4
FGQGTRLEIK

SEQ ID NO: 163 - protein, 10 aa, Artificial Sequence
  PR004275|pHBM005296-VL|L-FR4
FGPGTKVDIK

SEQ ID NO: 164 - protein, 10 aa, Artificial Sequence
  L-FR4
FGQGTKLEIK

SEQ ID NO: 165 - protein, 10 aa, Artificial Sequence
  PR004970|pHBM006122-VL|L-FR4
FGQGTKVEIK

SEQ ID NO: 166 - protein, 10 aa, Artificial Sequence
  PR005124|pHBM006275-VL|L-FR4; PR005127|pHBM006275-VL|L-FR4
FGQGTKVDIK

SEQ ID NO: 167 - protein, 123 aa, Artificial Sequence
  PR004120|pHBM005087-VH|VH
EVQLVESGGGLVQPKGSLKLSCAASGFTFNTNAMNWVRQAPGKGLEWVARIRSKMNNYATYYADSVKDRFTISRDDSQNMLYLQMNNLKTEDTAMYYCVRGKENGNYYAMDFWGQGTSVTVSA

SEQ ID NO: 168 - protein, 123 aa, Artificial Sequence
  PR004121|pHBM005088-VH|VH
EVQLVESGGGLVQPKGSLKLSCAASGFTFNTYAMNWVRQAPGKGLEWVARIRSKSNNYATYYADSVKDRFTISRDDSQNMLYLQMNNLKTEDTAMYYCVRGKENGNYYAMDFWGQGTSVTVSS

SEQ ID NO: 169 - protein, 123 aa, Artificial Sequence
  PR004122|pHBM005089-VH|VH; PR004249|pHBM005373-VH|VH
EVQLVETGGGLVQPKGSLKLSCAASGFTFNTNAMNWVRQAPGKGLEWVARIRSKSNNYATYYADSVKDRFTISRDDSQSMLYLQMNNLKTEDTAMYYCVRGKENGNYYAMDFWGQGTSVTVSS

SEQ ID NO: 170 - protein, 123 aa, Artificial Sequence
  PR004123|pHBM005090-VH|VH
EVQLVESGGGLVQPKGSLKLSCAASEFTFNTYAMNWVRQAPGKGLEWVARIRTKSNNFATYYADSVKDRFTISRDDSQSMLFLQMNNLKTEDTAMYYCVRGKENGNYYAMDFWGQGTSVTVSA

SEQ ID NO: 171 - protein, 123 aa, Artificial Sequence
  PR004124|pHBM005091-VH|VH
EVKVEESGGGLVQPGGSMKLSCAASGFTFNTYAMNWVRQAPGKGLEWVARIRSKSNNYATYYADSVKDRFTISRDDSQSMLYLQMNNLKTEDTAMYYCVRGKDYGNYYAMDFWGQGTSLTVSS

SEQ ID NO: 172 - protein, 123 aa, Artificial Sequence
  PR004125|pHBM005092-VH|VH; PR004128|pHBM005092-VH|VH; PR004250|pHBM005374-VH|VH; PR004251|pHBM005374-VH|VH; PR004324|pHBM005374-VH|VH; PR004325|pHBM005374-VH|VH; PR004339|pHBM005374-VH|VH; PR004340|pHBM005374-VH|VH; PR004342|pHBM005374-VH|VH; PR004343|pHBM005374-VH|VH; PR004344|pHBM005374-VH|VH; PR004345|pHBM005374-VH|VH; PR004346|pHBM005374-VH|VH; PR005170|pHBM005092-VH|VH; PR005171|pHBM005092-VH|VH; PR005172|pHBM005092-VH|VH
EVQLVESGGGLVQPKGSLKLSCAASGFTFNTYAMNWVRQAPGKGLEWVARIRSKSNNYATYYADSVKDRFTISRDDSQSMLYLQMNNLKTEDTAMYYCVRGKENGNYYAMDFWGQGTSVTVSA

SEQ ID NO: 173 - protein, 123 aa, Artificial Sequence
  PR004126|pHBM005093-VH|VH
EVQLVESGGGLVQPKGSLKLSCAASGFTFSTNAMNWVRQAPGKGLEWVGRIRSKSNNYATYYADSVKDRFTISRDDSQSMLYLQMNNLKTEDTAMYYCVRGKENGNYYAMDFWGQGTSVTVSA

SEQ ID NO: 174 - protein, 123 aa, Artificial Sequence
  PR004127|pHBM005094-VH|VH
EVQLVETGGGLVQPKGSLKLSCAASGFTFNTNAMNWVRQAPGKGLEWVARIRSKSNNYATYYADSVKDRFTISRDDSQNMLYLQMNNLKTEDTAMYYCVRGKENGNYYAMDFWGQGTSVTVSS

SEQ ID NO: 175 - protein, 123 aa, Artificial Sequence
  PR004129|pHBM005095-VH|VH
EVQLVESGGGLVQPKGSLKLSCAASGFTFNTYAMNWVRQAPGKGLEWVARIRSKSNNYATYYADSVKDRFTISRDDSQSMLYLQMNNLKTEDTAMYYCVRGKDYGNYYAMDYWGQGTSVTVSS

SEQ ID NO: 176 - protein, 123 aa, Artificial Sequence
  PR004130|pHBM005096-VH|VH
EVQLVESGGGLVQFKGSLKLSCGTSGFTFNTYAMNWVRQAPGKGLEWVARIRSKSNNYATFYADSVKDRFTISRDDSQNMLYLQMNNLKTEDTAMYYCVRGKENGNYYAMDFWGQGTSVTVSS

SEQ ID NO: 177 - protein, 123 aa, Artificial Sequence
  PR004131|pHBM005097-VH|VH; PR004252|pHBM005375-VH|VH
EVQLVESGGGLVQPKGSLKLSCAASGFTFNTYAMNWVRQAPGKGLEWVARIRSKSNNYATYYADSVKDRFTISRDDSQSMLYLQMNNLKTEDTAMYYCVRGKENGNYYAMDYWGQGTSVTVSS

SEQ ID NO: 178 - protein, 114 aa, Artificial Sequence
  PR004264|pHBM005401-VH|VH
EVQLVESGGGLVQPGGSLRLSCAASGFTFSSYAMSWVRQAPGKGLEWVSAISGSGGSTYYADSVKGRFTISRDNSKNTLYLQMNSLRAEDTAVYYCATQGFDYWGQGTLVTVSS

SEQ ID NO: 179 - protein, 120 aa, Artificial Sequence
  PR004265|pHBM005403-VH|VH
EVQLVESGGGLVQPGGSRKLSCAASGFTFSSFGMHWVRQVPEKGLEWVAYISSGSRTIYYTDTVKGRFTISRDNPKNTLFLQMTSLRSEDTAIYYCVRGGLRPYWYFDVWGAGTTVTVSA

SEQ ID NO: 180 - protein, 119 aa, Artificial Sequence
  PR004275|pHBM005295-VH|VH
EVQLVESGGGLVQPGGSLRLSCAASGFTFSSYAMSWVRQAPGKGLEWVSAISGSGGSTYYADSVKGRFTISRDNSKNTLYLQMNSLRAEDTAVYYCARRWGKGGLFDYWGQGTLVTVSS

SEQ ID NO: 181 - protein, 123 aa, Artificial Sequence
  PR004326|pHBM005430-VH|VH
EVQLVESGGGLVQPKGSLKLSCAASGFTFNTYAMNWVRQAPGKGLEWVARIRSKSNNYATYYADSVKDRFTISRDDSQSMLYLQMNNLKTEDTAMYYCVRGKENANYYAMDFWGQGTSVTVSA

SEQ ID NO: 182 - protein, 123 aa, Artificial Sequence
  PR004327|pHBM005431-VH|VH
EVQLVESGGGLVQPKGSLKLSCAASGFTFQTYAMNWVRQAPGKGLEWVARIRSKSNNYATYYADSVKDRFTISRDDSQSMLYLQMNNLKTEDTAMYYCVRGKENGNYYAMDFWGQGTSVTVSA

SEQ ID NO: 183 - protein, 123 aa, Artificial Sequence
  PR004328|pHBM005432-VH|VH
EVQLVESGGGLVQPKGSLKLSCAASGFTFSTYAMNWVRQAPGKGLEWVARIRSKSNNYATYYADSVKDRFTISRDDSQSMLYLQMNNLKTEDTAMYYCVRGKENGNYYAMDFWGQGTSVTVSA

SEQ ID NO: 184 - protein, 123 aa, Artificial Sequence
  PR004329|pHBM005433-VH|VH
EVQLVESGGGLVQPKGSLKLSCAASGFTFNTYAMNWVRQAPGKGLEWVARIRSKSNNYATYYADSVKDRFTISRDDSQSMLYLQMNNLKTEDTAMYYCVRGKEQGNYYAMDFWGQGTSVTVSA

SEQ ID NO: 185 - protein, 123 aa, Artificial Sequence
  PR004330|pHBM005435-VH|VH; PR004519|pHBM005435-VH|VH; PR004522|pHBM005435-VH|VH; PR004525|pHBM005435-VH|VH; PR004669|pHBM005793-VH|VH
EVQLVESGGGLVKPGGSLRLSCAASGFTFNTYAMNWVRQAPGKGLEWVGRIRSKSNNYATYYADSVKDRFTISRDDSKSTLYLQMNSLKTEDTAVYYCVRGKENGNYYAMDFWGQGTTVTVSS

SEQ ID NO: 186 - protein, 123 aa, Artificial Sequence
  PR004331|pHBM005436-VH|VH
EVQLVESGGGLVKPGGSLRLSCAASGFTFNTNAMNWVRQAPGKGLEWVGRIRSKSNNYATYYADSVKDRFTISRDDSKSTLYLQMNSLKTEDTAVYYCVRGKENGNYYAMDFWGQGTTVTVSS

SEQ ID NO: 187 - protein, 123 aa, Artificial Sequence
  PR004332|pHBM005437-VH|VH
EVQLVESGGGLVKPGGSLRLSCAASGFTFNTYAMNWVRQAPGKGLEWVGRIRSKSNNYATYYADSVKDRFTISRDDSKSTLYLQMNSLKTEDTAVYYCVRGKENGNYYAMDYWGQGTTVTVSS

SEQ ID NO: 188 - protein, 123 aa, Artificial Sequence
  PR004333|pHBM005439-VH|VH; PR004520|pHBM005439-VH|VH; PR004523|pHBM005439-VH|VH; PR004526|pHBM005439-VH|VH; PR004668|pHBM005792-VH|VH
EVQLVESGGGLVQPGGSLRLSCAASGFTFNTYAMNWVRQAPGKGLEWVSRIRSKSNNYATYYADSVKDRFTISRDDSKSTLYLQMNSLRAEDTAVYYCVRGKENGNYYAMDFWGQGTTVTVSS

SEQ ID NO: 189 - protein, 123 aa, Artificial Sequence
  PR004334|pHBM005440-VH|VH
EVQLVESGGGLVQPGGSLRLSCAASGFTFNTNAMNWVRQAPGKGLEWVSRIRSKSNNYATYYADSVKDRFTISRDDSKSTLYLQMNSLRAEDTAVYYCVRGKENGNYYAMDFWGQGTTVTVSS

SEQ ID NO: 190 - protein, 123 aa, Artificial Sequence
  PR004335|pHBM005441-VH|VH
EVQLVESGGGLVQPGGSLRLSCAASGFTFNTYAMNWVRQAPGKGLEWVSRIRSKSNNYATYYADSVKDRFTISRDDSKSTLYLQMNSLRAEDTAVYYCVRGKENGNYYAMDYWGQGTTVTVSS

SEQ ID NO: 191 - protein, 123 aa, Artificial Sequence
  PR004336|pHBM005443-VH|VH; PR004521|pHBM005443-VH|VH; PR004524|pHBM005443-VH|VH; PR004527|pHBM005443-VH|VH
EVQLVESGGGLVQPGGSLKLSCAASGFTFNTYAMNWVRQASGKGLEWVGRIRSKSNNYATYYADSVKDRFTISRDDSKSTLYLQMNSLKTEDTAVYYCVRGKENGNYYAMDFWGQGTTVTVSS

SEQ ID NO: 192 - protein, 123 aa, Artificial Sequence
  PR004337|pHBM005444-VH|VH
EVQLVESGGGLVQPGGSLKLSCAASGFTFNTNAMNWVRQASGKGLEWVGRIRSKSNNYATYYADSVKDRFTISRDDSKSTLYLQMNSLKTEDTAVYYCVRGKENGNYYAMDFWGQGTTVTVSS

SEQ ID NO: 193 - protein, 123 aa, Artificial Sequence
  PR004338|pHBM005445-VH|VH
EVQLVESGGGLVQPGGSLKLSCAASGFTFNTYAMNWVRQASGKGLEWVGRIRSKSNNYATYYADSVKDRFTISRDDSKSTLYLQMNSLKTEDTAVYYCVRGKENGNYYAMDYWGQGTTVTVSS

SEQ ID NO: 194 - protein, 123 aa, Artificial Sequence
  PR004660|pHBM005788-VH|VH; PR004662|pHBM005788-VH|VH
EVQLVESGGGLVQPGGSLRLSCAASGFTFSTYAMNWVRQAPGKGLEWVSRIRSKSNNYATYYADSVKDRFTISRDDSKSTLYLQMNSLRAEDTAVYYCVRGKENANYYAMDFWGQGTTVTVSS

SEQ ID NO: 195 - protein, 123 aa, Artificial Sequence
  PR004661|pHBM005789-VH|VH; PR004663|pHBM005789-VH|VH
EVQLVESGGGLVQPGGSLRLSCAASGFTFSTYAMNWVRQAPGKGLEWVSRIRSKSNNYATYYADSVKDRFTISRDDSKSTLYLQMNSLRAEDTAVYYCVRGKEQGNYYAMDFWGQGTTVTVSS

SEQ ID NO: 196 - protein, 123 aa, Artificial Sequence
  PR004664|pHBM005786-VH|VH; PR004666|pHBM005786-VH|VH; PR005565|pHBM006805-VH|VH; PR005750|pHBM007021-VH|VH
EVQLVESGGGLVKPGGSLRLSCAASGFTFSTYAMNWVRQAPGKGLEWVGRIRSKSNNYATYYADSVKDRFTISRDDSKSTLYLQMNSLKTEDTAVYYCVRGKENANYYAMDFWGQGTTVTVSS

SEQ ID NO: 197 - protein, 123 aa, Artificial Sequence
  PR004665|pHBM005787-VH|VH; PR004667|pHBM005787-VH|VH
EVQLVESGGGLVKPGGSLRLSCAASGFTFSTYAMNWVRQAPGKGLEWVGRIRSKSNNYATYYADSVKDRFTISRDDSKSTLYLQMNSLKTEDTAVYYCVRGKEQGNYYAMDFWGQGTTVTVSS

SEQ ID NO: 198 - protein, 115 aa, Artificial Sequence
  PR004970|pHBM006115-VH|VH
EVQLVESGGGLVQPGGSLRLSCAASGFTFSSYWMSWVPQAPGKGLEWVANIKQDGSAKFYVDSVKGRFTISRDNAKNSLYLQMNSLRAEDTAVYYCARSWGFAYWGQGTLVTVSS

SEQ ID NO: 199 - protein, 127 aa, Artificial Sequence
  PR004974|pHBM006117-VH|VH; PR005293|pHBM006504-VH|VH
QITLKESGPTLVKPTQTLTLTCTFSGFSLSTSGVGVGWIRQPPGKALEWLALIYWNDDKRYSPSLKSRLTITKDTSKNQVVLTMTNMDPVDTATYYCAHRRLRYSGRYYYYYGTDVWGQGTTVTVSS

SEQ ID NO: 200 - protein, 122 aa, Artificial Sequence
  PR005124|pHBM006274-VH|VH; PR005127|pHBM006280-VH|VH
QVQLVESGGGVVQPGRSLRLSCVASGFTFSSYGMHWVRQAPGKGLEWVAVIWHDGSNIFYADSVKGRFTISRDNSKNTLYLQMNSLRAEDTAVYWCARHRRSDYWYYGMDVWGQGTTVTVSS

SEQ ID NO: 201 - protein, 124 aa, Artificial Sequence
  PR005125|pHBM006276-VH|VH; PR005128|pHBM006281-VH|VH
QVQLVESGGGVVQPGRSLRLSCAASGFTFSSYGMHWVRQVPGKGLEWVAVIWYDGSKKYYADSVKGRFTISRDNSKNTLYLQMNSLRAEDTAVYYCARGGFYYGSGNYSLFDYWGQGTLVTVSS

SEQ ID NO: 202 - protein, 123 aa, Artificial Sequence
  PR005329|pHBM006537-VH|VH; PR005332|pHBM006540-VH|VH
EVKLLESGGGLVQPKGSLKLSCAASGFTFNTYAMNWVRQAPGKGLEWVARIRTKSNNYATYYADSVKDRFTISRDDSHSMLYLQMNNLKTEDTAMYYCVRGKDNGNYYAMDFWGQGTSVTVSA

SEQ ID NO: 203 - protein, 123 aa, Artificial Sequence
  PR005330|pHBM006538-VH|VH; PR005333|pHBM006541-VH|VH
EVKLVESGGGLVQPGGSRKLSCAASGFTFNTYAMNWVRQAPGKGLEWVARIRSKSNNYATYYADSVKDRFTISRDDSQSMLYLQMNNLKTEDTAMYYCVRGKDYGNYYAMDFWGQGTSVTVSS

SEQ ID NO: 204 - protein, 115 aa, Artificial Sequence
  PR005331|pHBM006539-VH|VH; PR005336|pHBM006544-VH|VH
EVQLVESGGGLVQPGGSLRLSCAASGFTFSNYWLSWVRQAPGKGLEWVANIKQDGSAKYYVDSVKGRFTISRDNAKNSLYLQMNSLRAEDTAVYYCVRNWGFDYWGQGTLVTVSS

SEQ ID NO: 205 - protein, 115 aa, Artificial Sequence
  PR005335|pHBM006543-VH|VH
QVQLVQSGGGLVQPGGSLRLSCTASGFTFSYYWLSWVRQAPGKGLEWVANIKQDGSTTYYVDSVKGRFTISRDNAKNSLYLQMNSLRAEDTAVYYCARNWGFDYWGQGTLVTVSS

SEQ ID NO: 206 - protein, 123 aa, Artificial Sequence
  PR005751|pHBM007019-VH|VH; PR006154|pHBM007001-VH|VH; PR006272|pHBM007521-VH|VH
EVQLVESGGGLVKPGGSLRLSCAASGFTFSTYAMNWVRQAPGKGLEWVGRIRSKSNNYATYYADSVKDRFTISRDDSKSTLYLQMNSLKTEDTAVYYCVRGKEHGNYYAMDFWGQGTTVTVSS

SEQ ID NO: 207 - protein, 123 aa, Artificial Sequence
  PR005752|pHBM007009-VH|VH; PR006155|pHBM006991-VH|VH; PR006276|pHBM007525-VH|VH
EVQLVESGGGLVKPGGSLRLSCAASGFTFSTYAMNWVRQAPGKGLEWVGRIRSKSNYYATYYADSVKDRFTISRDDSKSTLYLQMNSLKTEDTAVYYCVRGKEHGNYYAMDFWGQGTTVTVSS

SEQ ID NO: 208 - protein, 123 aa, Artificial Sequence
  PR005753|pHBM007020-VH|VH; PR006156|pHBM007002-VH|VH; PR006273|pHBM007522-VH|VH
EVQLVESGGGLVKPGGSLRLSCAASGFTFSTYAMNWVRQAPGKGLEWVGRIRSKSNNYATYYADSVKDRFTISRDDSKSTLYLQMNSLKTEDTAVYYCVRGKEIGNYYAMDFWGQGTTVTVSS

SEQ ID NO: 209 - protein, 123 aa, Artificial Sequence
  PR005754|pHBM007010-VH|VH; PR006157|pHBM006992-VH|VH; PR006277|pHBM007526-VH|VH
EVQLVESGGGLVKPGGSLRLSCAASGFTFSTYAMNWVRQAPGKGLEWVGRIRSKSNYYATYYADSVKDRFTISRDDSKSTLYLQMNSLKTEDTAVYYCVRGKEIGNYYAMDFWGQGTTVTVSS

SEQ ID NO: 210 - protein, 123 aa, Artificial Sequence
  PR005763|pHBM007005-VH|VH; PR006161|pHBM006987-VH|VH; PR006274|pHBM007523-VH|VH
EVQLVESGGGLVKPGGSLRLSCAASGFTFSTYAMNWVRQAPGKGLEWVGRIRSKSNYYATYYADSVKDRFTISRDDSKSTLYLQMNSLKTEDTAVYYCVRGKEHGKYYAMDFWGQGTTVTVSS

SEQ ID NO: 211 - protein, 123 aa, Artificial Sequence
  PR005787|pHBM007006-VH|VH; PR006166|pHBM006988-VH|VH; PR006275|pHBM007524-VH|VH
EVQLVESGGGLVKPGGSLRLSCAASGFTFSTYAMNWVRQAPGKGLEWVGRIRSKSNYYATYYADSVKDRFTISRDDSKSTLYLQMNSLKTEDTAVYYCVRGKEIGKYYAMDFWGQGTTVTVSS

SEQ ID NO: 212 - protein, 112 aa, Artificial Sequence
  PR004120|pHBM005098-VL|VL
DIVMTQAATSVLVTPGESVSISCRSSKSLLYSNGNTYLYWFLQRPGQSPQLLIYRMSNLASGVPDRFSGSGSGTAFTLRISRVEAEDVGVYYCMQHLEYPFTFGGGTKLEIK

SEQ ID NO: 213 - protein, 112 aa, Artificial Sequence
  PR004121|pHBM005099-VL|VL
DIVITQAAPSVPVTPGESVSISCRSSKSLLHSNGNTYLYWFLQRPGQSPQLLIYRMSNLASGVPDRFSGSGSGTAFTLRISRVEAEDVGVYYCMQHLEYPFTFGGGTKLEMK

SEQ ID NO: 214 - protein, 112 aa, Artificial Sequence
  PR004122|pHBM005100-VL|VL; PR004249|pHBM005100-VL|VL
DIVMTQAAPSVPVTPGESVSISCRSSKSLLHSNGNTYLYWFLQRPGQSPQLLIYRMSNLASGVPDRFSGSGSGTAFTLRISRVEAEDVGVYYCMQHLEYPLTFGAGTKLELK

SEQ ID NO: 215 - protein, 112 aa, Artificial Sequence
  PR004123|pHBM005101-VL|VL
DIVMTQAAPSVPVTPGESVSISCRSSKSLLHSNGNTYLYWFLQRPGQSPQLLIYRMSNLASGVPDRFSGSGSGTAFTLRISRVEAEDVGVYYCMQHLEYPFTFGGGTKLELK

SEQ ID NO: 216 - protein, 112 aa, Artificial Sequence
  PR004124|pHBM005102-VL|VL
DIVMTQDELSNPVTSGESVSISCRSSKSLLHSNGNTYLYWFLQRPGQSPQLLIYRMSNLASGVPDRFSGSGSGTAFTLRISRVEAEDVGVYYCMQHLEYPFTFGGGTKLELK

SEQ ID NO: 217 - protein, 112 aa, Artificial Sequence
  PR004125|pHBM005103-VL|VL; PR004250|pHBM005103-VL|VL
DIVMTQAAPSVPVTPGESVSISCRSSKSLLHSNGNTYLYWFLQRPGQSPQLLIYRMSNLASGVPDRFSGSGSGTAFTLRISRVEAEDVGVYYCMQHLEYPLTFGAGTKLEMK

SEQ ID NO: 218 - protein, 112 aa, Artificial Sequence
  PR004126|pHBM005104-VL|VL
DIVITQAAPSVPVTPGESVSISCRSSKSLLHSNGNTYLYWFLQRPGQSPQLLIYRMSNLASGVPDRFSGSGSGTAFTLRISRVEAEDVGVYYCMQHLEYPFTFGAGTKLELK

SEQ ID NO: 219 - protein, 112 aa, Artificial Sequence
  PR004127|pHBM005105-VL|VL
DIVMTQAATSVLVTPGESVSISCRSSKSLLYSNGNTYLYWFLQRPGQSPQLLIYRMSNLASGVPDRFSGSGSGTAFTLRISRVEAEDVGVYYCMQHLEYPFTFGGGTKLEMK

SEQ ID NO: 220 - protein, 112 aa, Artificial Sequence
  PR004128|pHBM005106-VL|VL; PR004251|pHBM005106-VL|VL; PR004326|pHBM005106-VL|VL; PR004327|pHBM005106-VL|VL; PR004328|pHBM005106-VL|VL; PR004329|pHBM005106-VL|VL; PR004330|pHBM005106-VL|VL; PR004331|pHBM005106-VL|VL; PR004332|pHBM005106-VL|VL; PR004333|pHBM005106-VL|VL; PR004334|pHBM005106-VL|VL; PR004335|pHBM005106-VL|VL; PR004336|pHBM005106-VL|VL; PR004337|pHBM005106-VL|VL; PR004338|pHBM005106-VL|VL
DIVMTQAAPSVPVTPGESVSISCRSSKSLLHSNGKIYLYWFLQRPGQSPQLLIYRMSNLASGVPDRFSGSGSGTAFTLRISRVEAEDVGVYYCMQHLEYPLTFGAGTKLEIK

SEQ ID NO: 221 - protein, 112 aa, Artificial Sequence
  PR004129|pHBM005107-VL|VL
DILLTQSPAILSVSPGERVSFSCRSSKSLLHSNGNTYLYWFLQRPGQSPQLLIYRMSNLASGVPDRFSGSGSGTAFTLRISRVEAEDVGVYYCMQHLEYPFTFGSGTKLEIN

SEQ ID NO: 222 - protein, 112 aa, Artificial Sequence
  PR004130|pHBM005108-VL|VL
DIVMTQAAPSVPVTPGESVSISCRSSKSLLHSNGNTYLYWFLQRPGQSPQLLIYRMSNLASGVPDRFSGSGSGTAFTLRISRVEAEDVGVYYCMQHLEYPFTFGSGTKLEIK

SEQ ID NO: 223 - protein, 112 aa, Artificial Sequence
  PR004131|pHBM005109-VL|VL; PR004252|pHBM005109-VL|VL
DIVMTQAAPSVPVTPGESVSISCRSNKSLLHSNGNTYLYWFLQRPGQSPQLLIYRMSNLASGVPDRFSGSGSGTAFTLRISRVEAEDVGVYYCMQHLEYPLTFGAGTKLEIK

SEQ ID NO: 224 - protein, 113 aa, Artificial Sequence
  PR004264|pHBM005402-VL|VL
DVVMTQSPLSLPVTLGQPASISCRSSQSLVYSDGNTYLNWFQQRPGQSPRRLIYKVSNRDSGVPDRFSGSGSGTDFTLKISRVEAEDVGVYYCMQGTHWPPITFGQGTRLEIK

SEQ ID NO: 225 - protein, 106 aa, Artificial Sequence
  PR004265|pHBM005404-VL|VL
DIVLIQSPAIMSASPGEKVTISCSASSSVSYMYWYQQKPGSSPKPWIYRTSNLASGVPARFSGSGSGTSYSLTISRMEAEDAATYYCQQRSSYPPTFGAGTKLELK

SEQ ID NO: 226 - protein, 107 aa, Artificial Sequence
  PR004275|pHBM005296-VL|VL
DIQLTQSPSTLSASVGDRVTITCRASQSISSWLAWYQQKPGKAPKLLIYKASSLESGVPSRFSGSGSGTDFTLTISSLQPEDVATYYCQKYNSAPPTFGPGTKVDIK

SEQ ID NO: 227 - protein, 112 aa, Artificial Sequence
  PR004324|pHBM005456-VL|VL
DIVMTQAAPSVPVTPGESVSISCRSSKSLLHSNAKIYLYWFLQRPGQSPQLLIYRMSNLASGVPDRFSGSGSGTAFTLRISRVEAEDVGVYYCMQHLEYPLTFGAGTKLEIK

SEQ ID NO: 228 - protein, 112 aa, Artificial Sequence
  PR004325|pHBM005457-VL|VL
DIVMTQAAPSVPVTPGESVSISCRSSKSLLHSQGKIYLYWFLQRPGQSPQLLIYRMSNLASGVPDRFSGSGSGTAFTLRISRVEAEDVGVYYCMQHLEYPLTFGAGTKLEIK

SEQ ID NO: 229 - protein, 112 aa, Artificial Sequence
  PR004339|pHBM005447-VL|VL; PR004519|pHBM005447-VL|VL; PR004520|pHBM005447-VL|VL; PR004521|pHBM005447-VL|VL; PR004660|pHBM005447-VL|VL; PR004661|pHBM005447-VL|VL; PR004668|pHBM005447-VL|VL
DIVMTQSPLSLPVTPGEPASISCRSSKSLLHSNGKIYLYWFLQKPGQSPQLLIYRMSNLASGVPDRFSGSGSGTDFTLKISRVEAEDVGVYYCMQHLEYPLTFGQGTKLEIK

SEQ ID NO: 230 - protein, 112 aa, Artificial Sequence
  PR004340|pHBM005448-VL|VL; PR004522|pHBM005448-VL|VL; PR004523|pHBM005448-VL|VL; PR004524|pHBM005448-VL|VL
DIVMTQSPLSLPVTPGEPASISCRSSKSLLHSNGNTYLYWFLQKPGQSPQLLIYRMSNLASGVPDRFSGSGSGTDFTLKISRVEAEDVGVYYCMQHLEYPLTFGQGTKLEIK

SEQ ID NO: 231 - protein, 112 aa, Artificial Sequence
  PR004342|pHBM005450-VL|VL
DIVMTQSPLSLPVTPGEPASISCRSSKSLLHSNGNTYLYWFLQKPGQSPQLLIYRMSNLASGVPDRFSGSGSGTDFTLKISRVEAEDVGVYYCMQHLEYPFTFGQGTKLEIK

SEQ ID NO: 232 - protein, 112 aa, Artificial Sequence
  VL
DIVMTQSPLSLPVTLGQPASISCRSSKSLLHSNGKIYLYWFQQRPGQSPRLLIYRMSNLASGVPDRFSGSGSGTDFTLKISRVEAEDVGVYYCMQHLEYPLTFGQGTKLEIK

SEQ ID NO: 233 - protein, 112 aa, Artificial Sequence
  PR004344|pHBM005453-VL|VL
DIVMTQSPLSLPVTLGQPASISCRSSKSLLHSNGNTYLYWFQQRPGQSPRLLIYRMSNLASGVPDRFSGSGSGTDFTLKISRVEAEDVGVYYCMQHLEYPLTFGQGTKLEIK

SEQ ID NO: 234 - protein, 112 aa, Artificial Sequence
  PR004345|pHBM005454-VL|VL
DIVMTQSPLSLPVTLGQPASISCRSNKSLLHSNGNTYLYWFQQRPGQSPRLLIYRMSNLASGVPDRFSGSGSGTDFTLKISRVEAEDVGVYYCMQHLEYPLTFGQGTKLEIK

SEQ ID NO: 235 - protein, 112 aa, Artificial Sequence
  PR004346|pHBM005455-VL|VL
DIVMTQSPLSLPVTLGQPASISCRSSKSLLHSNGNTYLYWFQQRPGQSPRLLIYRMSNLASGVPDRFSGSGSGTDFTLKISRVEAEDVGVYYCMQHLEYPFTFGQGTKLEIK

SEQ ID NO: 236 - protein, 112 aa, Artificial Sequence
  PR004662|pHBM005790-VL|VL; PR004663|pHBM005790-VL|VL
DIVMTQSPLSLPVTPGEPASISCRSSKSLLHSNAKIYLYWFLQKPGQSPQLLIYRMSNLASGVPDRFSGSGSGTDFTLKISRVEAEDVGVYYCMQHLEYPLTFGQGTKLEIK

SEQ ID NO: 237 - protein, 112 aa, Artificial Sequence
  PR004666|pHBM005791-VL|VL; PR004667|pHBM005791-VL|VL; PR005565|pHBM005791-VL|VL; PR005750|pHBM005791-VL|VL; PR005751|pHBM005791-VL|VL; PR005752|pHBM005791-VL|VL; PR005753|pHBM005791-VL|VL; PR005754|pHBM005791-VL|VL; PR005763|pHBM005791-VL|VL; PR005787|pHBM005791-VL|VL; PR006154|pHBM005791-VL|VL; PR006155|pHBM005791-VL|VL; PR006156|pHBM005791-VL|VL; PR006157|pHBM005791-VL|VL; PR006161|pHBM005791-VL|VL; PR006166|pHBM005791-VL|VL; PR006272|pHBM005791-VL|VL; PR006273|pHBM005791-VL|VL; PR006274|pHBM005791-VL|VL; PR006275|pHBM005791-VL|VL; PR006276|pHBM005791-VL|VL; PR006277|pHBM005791-VL|VL
DIVMTQSPLSLPVTLGQPASISCRSSKSLLHSNAKIYLYWFQQRPGQSPRLLIYRMSNLASGVPDRFSGSGSGTDFTLKISRVEAEDVGVYYCMQHLEYPLTFGQGTKLEIK

SEQ ID NO: 238 - protein, 107 aa, Artificial Sequence
  PR004970|pHBM006122-VL|VL
DIQMTQSPSSLSASVGDRVTITCRASQGISNYLAWYQQKPGKVPKLLIYAASTLQSGVPSRFSGSGSGTDFTLTISSLQPEDVATYYCQKYNSAPWTFGQGTKVEIK

SEQ ID NO: 239 - protein, 107 aa, Artificial Sequence
  PR004974|pHBM006126-VL|VL; PR005293|pHBM006126-VL|VL
EIVMTQSPATLSVSPGERATLSCRASQSVSSNLVWYQQKPGQAPRLLIYGASIRATGIPARFSGSGSGTEFTLTISSLQSEDFAVYYCQQYNNWPYTFGQGTKLEIK

SEQ ID NO: 240 - protein, 112 aa, Artificial Sequence
  PR005124|pHBM006275-VL|VL; PR005127|pHBM006275-VL|VL
DVVMTQSPLSLPVTPGEPASISCRSSQSLLHSNGYNYLDWYLQKPGQSPQLLIYLGSNRASGVPDRFSGSGSGTDFTLKISRVEAEDVGVYYCMQALQTPYTFGQGTKVDIK

SEQ ID NO: 241 - protein, 111 aa, Artificial Sequence
  PR005125|pHBM006277-VL|VL; PR005128|pHBM006277-VL|VL
DIVMTQSPLSLSVTLGQPASISCRSSQSLVFSNGNTYLNWFQQRPGQSPRRLIYKVSKRDSGVPDRFSGSGSGTDFTLKISRVEAEDVGVYYCMQGTHWITFGQGTRLEIK

SEQ ID NO: 242 - protein, 112 aa, Artificial Sequence
  PR005170|pHBM006323-VL|VL
DIVMTQAAPSVPVTPGESVSISCRSSKSLLHSNGKIYLYWFLQRPGQSPQLLIYRMSNLASGVPDRFSGSGSGTAFTLRISRVEAEDVGVYYCMQHLEYPITFGAGTKLEIK

SEQ ID NO: 243 - protein, 112 aa, Artificial Sequence
  PR005171|pHBM006324-VL|VL
DIVMTQAAPSVPVTPGESVSISCRSSKSLLHSNGKIYLYWFLQRPGQSPQLLIYRMSNLASGVPDRFSGSGSGTAFTLRISRVEAEDVGVYYCMQHLEYPMTFGAGTKLEIK

SEQ ID NO: 244 - protein, 112 aa, Artificial Sequence
  PR005172|pHBM006325-VL|VL
DIVMTQAAPSVPVTPGESVSISCRSSKSLLHSNGKIYLYWFLQRPGQSPQLLIYRMSNLASGVPDRFSGSGSGTAFTLRISRVEAEDVGVYYCMQHLEYPVTFGAGTKLEIK

SEQ ID NO: 245 - protein, 112 aa, Artificial Sequence
  PR005329|pHBM006545-VL|VL; PR005332|pHBM006545-VL|VL
DIVMTQAAPSVPVTPGESVSISCRSSKSLLHSNGNTYLYWFLQRPGQSPQLLIYRMSNLASGVPDRFSSSGSGTDFTLRISRVEAEDVGVYYCMQHLEYPFTFGAGTKLEIK

SEQ ID NO: 246 - protein, 112 aa, Artificial Sequence
  PR005330|pHBM006546-VL|VL; PR005333|pHBM006546-VL|VL
DIVMTQAATSVLVTPGESVSISCRSSKSLLYSNGNTYLYWFLQRPGQSPQLLIYRMSNLASGVPDRFSGSGSGTAFTLRISRVEAEDVGVYYCMQHLEYPFTFGGGTKLELK

SEQ ID NO: 247 - protein, 112 aa, Artificial Sequence
  PR005331|pHBM006549-VL|VL; PR005336|pHBM006549-VL|VL
DIVMTQSPLSLPVTLGQPASISCRSSQSLVYSNGNTYLNWFQQRPGQSPRRLIYKVSNRDSGVPDRFSGSGSGTDFTLKISRVEAEDVGVYYCMQGTHWPITFGQGTRLEIK

SEQ ID NO: 248 - protein, 112 aa, Artificial Sequence
  PR005335|pHBM006548-VL|VL
DVVMTQSPLSLPVTLGQPASISCRSSQSLVYSNGNTYLNWFQQRPGQSPRRLIYKVSNRDSGVPDRFSGSGSGTDFTLKISRVEAEDVGVYYCMQGTHWPITFGQGTRLEIK

SEQ ID NO: 249 - protein, 453 aa, Artificial Sequence
  PR004120|pHBM005087|HC
EVQLVESGGGLVQPKGSLKLSCAASGFTFNTNAMNWVRQAPGKGLEWVARIRSKMNNYATYYADSVKDRFTISRDDSQNMLYLQMNNLKTEDTAMYYCVRGKENGNYYAMDFWGQGTSVTVSAASTKGPSVFPLAPSSKSTSGGTAALGCLVKDYFPEPVTVSWNSGALTSGVHTFPAVLQSSGLYSLSSVVTVPSSSLGTQTYICNVNHKPSNTKVDKKVEPKSCDKTHTCPPCPAPELLGGPSVFLFPPKPKDTLMISRTPEVTCVVVDVSHEDPEVKFNWYVDGVEVHNAKTKPREEQYNSTYRVVSVLTVLHQDWLNGKEYKCKVSNKALPAPIEKTISKAKGQPREPQVYTLPPSREEMTKNQVSLTCLVKGFYPSDIAVEWESNGQPENNYKTTPPVLDSDGSFFLYSKLTVDKSRWQQGNVFSCSVMHEALHNHYTQKSLSLSPGK

SEQ ID NO: 250 - protein, 453 aa, Artificial Sequence
  PR004121|pHBM005088|HC
EVQLVESGGGLVQPKGSLKLSCAASGFTFNTYAMNWVRQAPGKGLEWVARIRSKSNNYATYYADSVKDRFTISRDDSQNMLYLQMNNLKTEDTAMYYCVRGKENGNYYAMDFWGQGTSVTVSSASTKGPSVFPLAPSSKSTSGGTAALGCLVKDYFPEPVTVSWNSGALTSGVHTFPAVLQSSGLYSLSSVVTVPSSSLGTQTYICNVNHKPSNTKVDKKVEPKSCDKTHTCPPCPAPELLGGPSVFLFPPKPKDTLMISRTPEVTCVVVDVSHEDPEVKFNWYVDGVEVHNAKTKPREEQYNSTYRVVSVLTVLHQDWLNGKEYKCKVSNKALPAPIEKTISKAKGQPREPQVYTLPPSREEMTKNQVSLTCLVKGFYPSDIAVEWESNGQPENNYKTTPPVLDSDGSFFLYSKLTVDKSRWQQGNVFSCSVMHEALHNHYTQKSLSLSPGK

SEQ ID NO: 251 - protein, 453 aa, Artificial Sequence
  PR004122|pHBM005089|HC
EVQLVETGGGLVQPKGSLKLSCAASGFTFNTNAMNWVRQAPGKGLEWVARIRSKSNNYATYYADSVKDRFTISRDDSQSMLYLQMNNLKTEDTAMYYCVRGKENGNYYAMDFWGQGTSVTVSSASTKGPSVFPLAPSSKSTSGGTAALGCLVKDYFPEPVTVSWNSGALTSGVHTFPAVLQSSGLYSLSSVVTVPSSSLGTQTYICNVNHKPSNTKVDKKVEPKSCDKTHTCPPCPAPELLGGPSVFLFPPKPKDTLMISRTPEVTCVVVDVSHEDPEVKFNWYVDGVEVHNAKTKPREEQYNSTYRVVSVLTVLHQDWLNGKEYKCKVSNKALPAPIEKTISKAKGQPREPQVYTLPPSREEMTKNQVSLTCLVKGFYPSDIAVEWESNGQPENNYKTTPPVLDSDGSFFLYSKLTVDKSRWQQGNVFSCSVMHEALHNHYTQKSLSLSPGK

SEQ ID NO: 252 - protein, 453 aa, Artificial Sequence
  PR004123|pHBM005090|HC
EVQLVESGGGLVQPKGSLKLSCAASEFTFNTYAMNWVRQAPGKGLEWVARIRTKSNNFATYYADSVKDRFTISRDDSQSMLFLQMNNLKTEDTAMYYCVRGKENGNYYAMDFWGQGTSVTVSAASTKGPSVFPLAPSSKSTSGGTAALGCLVKDYFPEPVTVSWNSGALTSGVHTFPAVLQSSGLYSLSSVVTVPSSSLGTQTYICNVNHKPSNTKVDKKVEPKSCDKTHTCPPCPAPELLGGPSVFLFPPKPKDTLMISRTPEVTCVVVDVSHEDPEVKFNWYVDGVEVHNAKTKPREEQYNSTYRVVSVLTVLHQDWLNGKEYKCKVSNKALPAPIEKTISKAKGQPREPQVYTLPPSREEMTKNQVSLTCLVKGFYPSDIAVEWESNGQPENNYKTTPPVLDSDGSFFLYSKLTVDKSRWQQGNVFSCSVMHEALHNHYTQKSLSLSPGK

SEQ ID NO: 253 - protein, 453 aa, Artificial Sequence
  PR004124|pHBM005091|HC
EVKVEESGGGLVQPGGSMKLSCAASGFTFNTYAMNWVRQAPGKGLEWVARIRSKSNNYATYYADSVKDRFTISRDDSQSMLYLQMNNLKTEDTAMYYCVRGKDYGNYYAMDFWGQGTSLTVSSASTKGPSVFPLAPSSKSTSGGTAALGCLVKDYFPEPVTVSWNSGALTSGVHTFPAVLQSSGLYSLSSVVTVPSSSLGTQTYICNVNHKPSNTKVDKKVEPKSCDKTHTCPPCPAPELLGGPSVFLFPPKPKDTLMISRTPEVTCVVVDVSHEDPEVKFNWYVDGVEVHNAKTKPREEQYNSTYRVVSVLTVLHQDWLNGKEYKCKVSNKALPAPIEKTISKAKGQPREPQVYTLPPSREEMTKNQVSLTCLVKGFYPSDIAVEWESNGQPENNYKTTPPVLDSDGSFFLYSKLTVDKSRWQQGNVFSCSVMHEALHNHYTQKSLSLSPGK

SEQ ID NO: 254 - protein, 453 aa, Artificial Sequence
  HC
EVQLVESGGGLVQPKGSLKLSCAASGFTFNTYAMNWVRQAPGKGLEWVARIRSKSNNYATYYADSVKDRFTISRDDSQSMLYLQMNNLKTEDTAMYYCVRGKENGNYYAMDFWGQGTSVTVSAASTKGPSVFPLAPSSKSTSGGTAALGCLVKDYFPEPVTVSWNSGALTSGVHTFPAVLQSSGLYSLSSVVTVPSSSLGTQTYICNVNHKPSNTKVDKKVEPKSCDKTHTCPPCPAPELLGGPSVFLFPPKPKDTLMISRTPEVTCVVVDVSHEDPEVKFNWYVDGVEVHNAKTKPREEQYNSTYRVVSVLTVLHQDWLNGKEYKCKVSNKALPAPIEKTISKAKGQPREPQVYTLPPSREEMTKNQVSLTCLVKGFYPSDIAVEWESNGQPENNYKTTPPVLDSDGSFFLYSKLTVDKSRWQQGNVFSCSVMHEALHNHYTQKSLSLSPGK

SEQ ID NO: 255 - protein, 453 aa, Artificial Sequence
  PR004126|pHBM005093|HC
EVQLVESGGGLVQPKGSLKLSCAASGFTFSTNAMNWVRQAPGKGLEWVGRIRSKSNNYATYYADSVKDRFTISRDDSQSMLYLQMNNLKTEDTAMYYCVRGKENGNYYAMDFWGQGTSVTVSAASTKGPSVFPLAPSSKSTSGGTAALGCLVKDYFPEPVTVSWNSGALTSGVHTFPAVLQSSGLYSLSSVVTVPSSSLGTQTYICNVNHKPSNTKVDKKVEPKSCDKTHTCPPCPAPELLGGPSVFLFPPKPKDTLMISRTPEVTCVVVDVSHEDPEVKFNWYVDGVEVHNAKTKPREEQYNSTYRVVSVLTVLHQDWLNGKEYKCKVSNKALPAPIEKTISKAKGQPREPQVYTLPPSREEMTKNQVSLTCLVKGFYPSDIAVEWESNGQPENNYKTTPPVLDSDGSFFLYSKLTVDKSRWQQGNVFSCSVMHEALHNHYTQKSLSLSPGK

SEQ ID NO: 256 - protein, 453 aa, Artificial Sequence
  PR004127|pHBM005094|HC
EVQLVETGGGLVQPKGSLKLSCAASGFTFNTNAMNWVRQAPGKGLEWVARIRSKSNNYATYYADSVKDRFTISRDDSQNMLYLQMNNLKTEDTAMYYCVRGKENGNYYAMDFWGQGTSVTVSSASTKGPSVFPLAPSSKSTSGGTAALGCLVKDYFPEPVTVSWNSGALTSGVHTFPAVLQSSGLYSLSSVVTVPSSSLGTQTYICNVNHKPSNTKVDKKVEPKSCDKTHTCPPCPAPELLGGPSVFLFPPKPKDTLMISRTPEVTCVVVDVSHEDPEVKFNWYVDGVEVHNAKTKPREEQYNSTYRVVSVLTVLHQDWLNGKEYKCKVSNKALPAPIEKTISKAKGQPREPQVYTLPPSREEMTKNQVSLTCLVKGFYPSDIAVEWESNGQPENNYKTTPPVLDSDGSFFLYSKLTVDKSRWQQGNVFSCSVMHEALHNHYTQKSLSLSPGK

SEQ ID NO: 257 - protein, 453 aa, Artificial Sequence
  PR004129|pHBM005095|HC
EVQLVESGGGLVQPKGSLKLSCAASGFTFNTYAMNWVRQAPGKGLEWVARIRSKSNNYATYYADSVKDRFTISRDDSQSMLYLQMNNLKTEDTAMYYCVRGKDYGNYYAMDYWGQGTSVTVSSASTKGPSVFPLAPSSKSTSGGTAALGCLVKDYFPEPVTVSWNSGALTSGVHTFPAVLQSSGLYSLSSVVTVPSSSLGTQTYICNVNHKPSNTKVDKKVEPKSCDKTHTCPPCPAPELLGGPSVFLFPPKPKDTLMISRTPEVTCVVVDVSHEDPEVKFNWYVDGVEVHNAKTKPREEQYNSTYRVVSVLTVLHQDWLNGKEYKCKVSNKALPAPIEKTISKAKGQPREPQVYTLPPSREEMTKNQVSLTCLVKGFYPSDIAVEWESNGQPENNYKTTPPVLDSDGSFFLYSKLTVDKSRWQQGNVFSCSVMHEALHNHYTQKSLSLSPGK

SEQ ID NO: 258 - protein, 453 aa, Artificial Sequence
  PR004130|pHBM005096|HC
EVQLVESGGGLVQFKGSLKLSCGTSGFTFNTYAMNWVRQAPGKGLEWVARIRSKSNNYATFYADSVKDRFTISRDDSQNMLYLQMNNLKTEDTAMYYCVRGKENGNYYAMDFWGQGTSVTVSSASTKGPSVFPLAPSSKSTSGGTAALGCLVKDYFPEPVTVSWNSGALTSGVHTFPAVLQSSGLYSLSSVVTVPSSSLGTQTYICNVNHKPSNTKVDKKVEPKSCDKTHTCPPCPAPELLGGPSVFLFPPKPKDTLMISRTPEVTCVVVDVSHEDPEVKFNWYVDGVEVHNAKTKPREEQYNSTYRVVSVLTVLHQDWLNGKEYKCKVSNKALPAPIEKTISKAKGQPREPQVYTLPPSREEMTKNQVSLTCLVKGFYPSDIAVEWESNGQPENNYKTTPPVLDSDGSFFLYSKLTVDKSRWQQGNVFSCSVMHEALHNHYTQKSLSLSPGK

SEQ ID NO: 259 - protein, 453 aa, Artificial Sequence
  PR004131|pHBM005097|HC
EVQLVESGGGLVQPKGSLKLSCAASGFTFNTYAMNWVRQAPGKGLEWVARIRSKSNNYATYYADSVKDRFTISRDDSQSMLYLQMNNLKTEDTAMYYCVRGKENGNYYAMDYWGQGTSVTVSSASTKGPSVFPLAPSSKSTSGGTAALGCLVKDYFPEPVTVSWNSGALTSGVHTFPAVLQSSGLYSLSSVVTVPSSSLGTQTYICNVNHKPSNTKVDKKVEPKSCDKTHTCPPCPAPELLGGPSVFLFPPKPKDTLMISRTPEVTCVVVDVSHEDPEVKFNWYVDGVEVHNAKTKPREEQYNSTYRVVSVLTVLHQDWLNGKEYKCKVSNKALPAPIEKTISKAKGQPREPQVYTLPPSREEMTKNQVSLTCLVKGFYPSDIAVEWESNGQPENNYKTTPPVLDSDGSFFLYSKLTVDKSRWQQGNVFSCSVMHEALHNHYTQKSLSLSPGK

SEQ ID NO: 260 - protein, 453 aa, Artificial Sequence
  PR004249|pHBM005373|HC
EVQLVETGGGLVQPKGSLKLSCAASGFTFNTNAMNWVRQAPGKGLEWVARIRSKSNNYATYYADSVKDRFTISRDDSQSMLYLQMNNLKTEDTAMYYCVRGKENGNYYAMDFWGQGTSVTVSSASTKGPSVFPLAPSSKSTSGGTAALGCLVKDYFPEPVTVSWNSGALTSGVHTFPAVLQSSGLYSLSSVVTVPSSSLGTQTYICNVNHKPSNTKVDKKVEPKSCDKTHTCPPCPAPELLGGPDVFLFPPKPKDTLMISRTPEVTCVVVDVSHEDPEVKFNWYVDGVEVHNAKTKPREEQYNSTYRVVSVLTVLHQDWLNGKEYKCKVSNKALPAPEEKTISKAKGQPREPQVYTLPPSREEMTKNQVSLTCLVKGFYPSDIAVEWESNGQPENNYKTTPPVLDSDGSFFLYSKLTVDKSRWQQGNVFSCSVMHEALHNHYTQKSLSLSPGK

SEQ ID NO: 261 - protein, 453 aa, Artificial Sequence
  HC
EVQLVESGGGLVQPKGSLKLSCAASGFTFNTYAMNWVRQAPGKGLEWVARIRSKSNNYATYYADSVKDRFTISRDDSQSMLYLQMNNLKTEDTAMYYCVRGKENGNYYAMDFWGQGTSVTVSAASTKGPSVFPLAPSSKSTSGGTAALGCLVKDYFPEPVTVSWNSGALTSGVHTFPAVLQSSGLYSLSSVVTVPSSSLGTQTYICNVNHKPSNTKVDKKVEPKSCDKTHTCPPCPAPELLGGPDVFLFPPKPKDTLMISRTPEVTCVVVDVSHEDPEVKFNWYVDGVEVHNAKTKPREEQYNSTYRVVSVLTVLHQDWLNGKEYKCKVSNKALPAPEEKTISKAKGQPREPQVYTLPPSREEMTKNQVSLTCLVKGFYPSDIAVEWESNGQPENNYKTTPPVLDSDGSFFLYSKLTVDKSRWQQGNVFSCSVMHEALHNHYTQKSLSLSPGK

SEQ ID NO: 262 - protein, 453 aa, Artificial Sequence
  PR004252|pHBM005375|HC
EVQLVESGGGLVQPKGSLKLSCAASGFTFNTYAMNWVRQAPGKGLEWVARIRSKSNNYATYYADSVKDRFTISRDDSQSMLYLQMNNLKTEDTAMYYCVRGKENGNYYAMDYWGQGTSVTVSSASTKGPSVFPLAPSSKSTSGGTAALGCLVKDYFPEPVTVSWNSGALTSGVHTFPAVLQSSGLYSLSSVVTVPSSSLGTQTYICNVNHKPSNTKVDKKVEPKSCDKTHTCPPCPAPELLGGPDVFLFPPKPKDTLMISRTPEVTCVVVDVSHEDPEVKFNWYVDGVEVHNAKTKPREEQYNSTYRVVSVLTVLHQDWLNGKEYKCKVSNKALPAPEEKTISKAKGQPREPQVYTLPPSREEMTKNQVSLTCLVKGFYPSDIAVEWESNGQPENNYKTTPPVLDSDGSFFLYSKLTVDKSRWQQGNVFSCSVMHEALHNHYTQKSLSLSPGK

SEQ ID NO: 263 - protein, 444 aa, Artificial Sequence
  PR004264|pHBM005401|HC
EVQLVESGGGLVQPGGSLRLSCAASGFTFSSYAMSWVRQAPGKGLEWVSAISGSGGSTYYADSVKGRFTISRDNSKNTLYLQMNSLRAEDTAVYYCATQGFDYWGQGTLVTVSSASTKGPSVFPLAPSSKSTSGGTAALGCLVKDYFPEPVTVSWNSGALTSGVHTFPAVLQSSGLYSLSSVVTVPSSSLGTQTYICNVNHKPSNTKVDKKVEPKSCDKTHTCPPCPAPELLGGPDVFLFPPKPKDTLMISRTPEVTCVVVDVSHEDPEVKFNWYVDGVEVHNAKTKPREEQYNSTYRVVSVLTVLHQDWLNGKEYKCKVSNKALPAPEEKTISKAKGQPREPQVYTLPPSREEMTKNQVSLTCLVKGFYPSDIAVEWESNGQPENNYKTTPPVLDSDGSFFLYSKLTVDKSRWQQGNVFSCSVMHEALHNHYTQKSLSLSPGK

SEQ ID NO: 264 - protein, 450 aa, Artificial Sequence
  PR004265|pHBM005403|HC
EVQLVESGGGLVQPGGSRKLSCAASGFTFSSFGMHWVRQVPEKGLEWVAYISSGSRTIYYTDTVKGRFTISRDNPKNTLFLQMTSLRSEDTAIYYCVRGGLRPYWYFDVWGAGTTVTVSAASTKGPSVFPLAPSSKSTSGGTAALGCLVKDYFPEPVTVSWNSGALTSGVHTFPAVLQSSGLYSLSSVVTVPSSSLGTQTYICNVNHKPSNTKVDKKVEPKSCDKTHTCPPCPAPELLGGPDVFLFPPKPKDTLMISRTPEVTCVVVDVSHEDPEVKFNWYVDGVEVHNAKTKPREEQYNSTYRVVSVLTVLHQDWLNGKEYKCKVSNKALPAPEEKTISKAKGQPREPQVYTLPPSREEMTKNQVSLTCLVKGFYPSDIAVEWESNGQPENNYKTTPPVLDSDGSFFLYSKLTVDKSRWQQGNVFSCSVMHEALHNHYTQKSLSLSPGK

SEQ ID NO: 265 - protein, 449 aa, Artificial Sequence
  PR004275|pHBM005295|HC
EVQLVESGGGLVQPGGSLRLSCAASGFTFSSYAMSWVRQAPGKGLEWVSAISGSGGSTYYADSVKGRFTISRDNSKNTLYLQMNSLRAEDTAVYYCARRWGKGGLFDYWGQGTLVTVSSASTKGPSVFPLAPSSKSTSGGTAALGCLVKDYFPEPVTVSWNSGALTSGVHTFPAVLQSSGLYSLSSVVTVPSSSLGTQTYICNVNHKPSNTKVDKKVEPKSCDKTHTCPPCPAPELLGGPSVFLFPPKPKDTLMISRTPEVTCVVVDVSHEDPEVKFNWYVDGVEVHNAKTKPREEQYNSTYRVVSVLTVLHQDWLNGKEYKCKVSNKALPAPIEKTISKAKGQPREPQVYTLPPSREEMTKNQVSLTCLVKGFYPSDIAVEWESNGQPENNYKTTPPVLDSDGSFFLYSKLTVDKSRWQQGNVFSCSVMHEALHNHYTQKSLSLSPGK

SEQ ID NO: 266 - protein, 453 aa, Artificial Sequence
  PR004326|pHBM005430|HC
EVQLVESGGGLVQPKGSLKLSCAASGFTFNTYAMNWVRQAPGKGLEWVARIRSKSNNYATYYADSVKDRFTISRDDSQSMLYLQMNNLKTEDTAMYYCVRGKENANYYAMDFWGQGTSVTVSAASTKGPSVFPLAPSSKSTSGGTAALGCLVKDYFPEPVTVSWNSGALTSGVHTFPAVLQSSGLYSLSSVVTVPSSSLGTQTYICNVNHKPSNTKVDKKVEPKSCDKTHTCPPCPAPELLGGPDVFLFPPKPKDTLMISRTPEVTCVVVDVSHEDPEVKFNWYVDGVEVHNAKTKPREEQYNSTYRVVSVLTVLHQDWLNGKEYKCKVSNKALPAPEEKTISKAKGQPREPQVYTLPPSREEMTKNQVSLTCLVKGFYPSDIAVEWESNGQPENNYKTTPPVLDSDGSFFLYSKLTVDKSRWQQGNVFSCSVMHEALHNHYTQKSLSLSPGK

SEQ ID NO: 267 - protein, 453 aa, Artificial Sequence
  PR004327|pHBM005431|HC
EVQLVESGGGLVQPKGSLKLSCAASGFTFQTYAMNWVRQAPGKGLEWVARIRSKSNNYATYYADSVKDRFTISRDDSQSMLYLQMNNLKTEDTAMYYCVRGKENGNYYAMDFWGQGTSVTVSAASTKGPSVFPLAPSSKSTSGGTAALGCLVKDYFPEPVTVSWNSGALTSGVHTFPAVLQSSGLYSLSSVVTVPSSSLGTQTYICNVNHKPSNTKVDKKVEPKSCDKTHTCPPCPAPELLGGPDVFLFPPKPKDTLMISRTPEVTCVVVDVSHEDPEVKFNWYVDGVEVHNAKTKPREEQYNSTYRVVSVLTVLHQDWLNGKEYKCKVSNKALPAPEEKTISKAKGQPREPQVYTLPPSREEMTKNQVSLTCLVKGFYPSDIAVEWESNGQPENNYKTTPPVLDSDGSFFLYSKLTVDKSRWQQGNVFSCSVMHEALHNHYTQKSLSLSPGK

SEQ ID NO: 268 - protein, 453 aa, Artificial Sequence
  PR004328|pHBM005432|HC
EVQLVESGGGLVQPKGSLKLSCAASGFTFSTYAMNWVRQAPGKGLEWVARIRSKSNNYATYYADSVKDRFTISRDDSQSMLYLQMNNLKTEDTAMYYCVRGKENGNYYAMDFWGQGTSVTVSAASTKGPSVFPLAPSSKSTSGGTAALGCLVKDYFPEPVTVSWNSGALTSGVHTFPAVLQSSGLYSLSSVVTVPSSSLGTQTYICNVNHKPSNTKVDKKVEPKSCDKTHTCPPCPAPELLGGPDVFLFPPKPKDTLMISRTPEVTCVVVDVSHEDPEVKFNWYVDGVEVHNAKTKPREEQYNSTYRVVSVLTVLHQDWLNGKEYKCKVSNKALPAPEEKTISKAKGQPREPQVYTLPPSREEMTKNQVSLTCLVKGFYPSDIAVEWESNGQPENNYKTTPPVLDSDGSFFLYSKLTVDKSRWQQGNVFSCSVMHEALHNHYTQKSLSLSPGK

SEQ ID NO: 269 - protein, 453 aa, Artificial Sequence
  PR004329|pHBM005433|HC
EVQLVESGGGLVQPKGSLKLSCAASGFTFNTYAMNWVRQAPGKGLEWVARIRSKSNNYATYYADSVKDRFTISRDDSQSMLYLQMNNLKTEDTAMYYCVRGKEQGNYYAMDFWGQGTSVTVSAASTKGPSVFPLAPSSKSTSGGTAALGCLVKDYFPEPVTVSWNSGALTSGVHTFPAVLQSSGLYSLSSVVTVPSSSLGTQTYICNVNHKPSNTKVDKKVEPKSCDKTHTCPPCPAPELLGGPDVFLFPPKPKDTLMISRTPEVTCVVVDVSHEDPEVKFNWYVDGVEVHNAKTKPREEQYNSTYRVVSVLTVLHQDWLNGKEYKCKVSNKALPAPEEKTISKAKGQPREPQVYTLPPSREEMTKNQVSLTCLVKGFYPSDIAVEWESNGQPENNYKTTPPVLDSDGSFFLYSKLTVDKSRWQQGNVFSCSVMHEALHNHYTQKSLSLSPGK

SEQ ID NO: 270 - protein, 453 aa, Artificial Sequence
  PR004330|pHBM005435|HC; PR004519|pHBM005435|HC; PR004522|pHBM005435|HC; PR004525|pHBM005435|HC
EVQLVESGGGLVKPGGSLRLSCAASGFTFNTYAMNWVRQAPGKGLEWVGRIRSKSNNYATYYADSVKDRFTISRDDSKSTLYLQMNSLKTEDTAVYYCVRGKENGNYYAMDFWGQGTTVTVSSASTKGPSVFPLAPSSKSTSGGTAALGCLVKDYFPEPVTVSWNSGALTSGVHTFPAVLQSSGLYSLSSVVTVPSSSLGTQTYICNVNHKPSNTKVDKKVEPKSCDKTHTCPPCPAPELLGGPDVFLFPPKPKDTLMISRTPEVTCVVVDVSHEDPEVKFNWYVDGVEVHNAKTKPREEQYNSTYRVVSVLTVLHQDWLNGKEYKCKVSNKALPAPEEKTISKAKGQPREPQVYTLPPSREEMTKNQVSLTCLVKGFYPSDIAVEWESNGQPENNYKTTPPVLDSDGSFFLYSKLTVDKSRWQQGNVFSCSVMHEALHNHYTQKSLSLSPGK

SEQ ID NO: 271 - protein, 453 aa, Artificial Sequence
  PR004331|pHBM005436|HC
EVQLVESGGGLVKPGGSLRLSCAASGFTFNTNAMNWVRQAPGKGLEWVGRIRSKSNNYATYYADSVKDRFTISRDDSKSTLYLQMNSLKTEDTAVYYCVRGKENGNYYAMDFWGQGTTVTVSSASTKGPSVFPLAPSSKSTSGGTAALGCLVKDYFPEPVTVSWNSGALTSGVHTFPAVLQSSGLYSLSSVVTVPSSSLGTQTYICNVNHKPSNTKVDKKVEPKSCDKTHTCPPCPAPELLGGPDVFLFPPKPKDTLMISRTPEVTCVVVDVSHEDPEVKFNWYVDGVEVHNAKTKPREEQYNSTYRVVSVLTVLHQDWLNGKEYKCKVSNKALPAPEEKTISKAKGQPREPQVYTLPPSREEMTKNQVSLTCLVKGFYPSDIAVEWESNGQPENNYKTTPPVLDSDGSFFLYSKLTVDKSRWQQGNVFSCSVMHEALHNHYTQKSLSLSPGK

SEQ ID NO: 272 - protein, 453 aa, Artificial Sequence
  PR004332|pHBM005437|HC
EVQLVESGGGLVKPGGSLRLSCAASGFTFNTYAMNWVRQAPGKGLEWVGRIRSKSNNYATYYADSVKDRFTISRDDSKSTLYLQMNSLKTEDTAVYYCVRGKENGNYYAMDYWGQGTTVTVSSASTKGPSVFPLAPSSKSTSGGTAALGCLVKDYFPEPVTVSWNSGALTSGVHTFPAVLQSSGLYSLSSVVTVPSSSLGTQTYICNVNHKPSNTKVDKKVEPKSCDKTHTCPPCPAPELLGGPDVFLFPPKPKDTLMISRTPEVTCVVVDVSHEDPEVKFNWYVDGVEVHNAKTKPREEQYNSTYRVVSVLTVLHQDWLNGKEYKCKVSNKALPAPEEKTISKAKGQPREPQVYTLPPSREEMTKNQVSLTCLVKGFYPSDIAVEWESNGQPENNYKTTPPVLDSDGSFFLYSKLTVDKSRWQQGNVFSCSVMHEALHNHYTQKSLSLSPGK

SEQ ID NO: 273 - protein, 453 aa, Artificial Sequence
  PR004333|pHBM005439|HC; PR004520|pHBM005439|HC; PR004523|pHBM005439|HC; PR004526|pHBM005439|HC
EVQLVESGGGLVQPGGSLRLSCAASGFTFNTYAMNWVRQAPGKGLEWVSRIRSKSNNYATYYADSVKDRFTISRDDSKSTLYLQMNSLRAEDTAVYYCVRGKENGNYYAMDFWGQGTTVTVSSASTKGPSVFPLAPSSKSTSGGTAALGCLVKDYFPEPVTVSWNSGALTSGVHTFPAVLQSSGLYSLSSVVTVPSSSLGTQTYICNVNHKPSNTKVDKKVEPKSCDKTHTCPPCPAPELLGGPDVFLFPPKPKDTLMISRTPEVTCVVVDVSHEDPEVKFNWYVDGVEVHNAKTKPREEQYNSTYRVVSVLTVLHQDWLNGKEYKCKVSNKALPAPEEKTISKAKGQPREPQVYTLPPSREEMTKNQVSLTCLVKGFYPSDIAVEWESNGQPENNYKTTPPVLDSDGSFFLYSKLTVDKSRWQQGNVFSCSVMHEALHNHYTQKSLSLSPGK

SEQ ID NO: 274 - protein, 453 aa, Artificial Sequence
  PR004334|pHBM005440|HC
EVQLVESGGGLVQPGGSLRLSCAASGFTFNTNAMNWVRQAPGKGLEWVSRIRSKSNNYATYYADSVKDRFTISRDDSKSTLYLQMNSLRAEDTAVYYCVRGKENGNYYAMDFWGQGTTVTVSSASTKGPSVFPLAPSSKSTSGGTAALGCLVKDYFPEPVTVSWNSGALTSGVHTFPAVLQSSGLYSLSSVVTVPSSSLGTQTYICNVNHKPSNTKVDKKVEPKSCDKTHTCPPCPAPELLGGPDVFLFPPKPKDTLMISRTPEVTCVVVDVSHEDPEVKFNWYVDGVEVHNAKTKPREEQYNSTYRVVSVLTVLHQDWLNGKEYKCKVSNKALPAPEEKTISKAKGQPREPQVYTLPPSREEMTKNQVSLTCLVKGFYPSDIAVEWESNGQPENNYKTTPPVLDSDGSFFLYSKLTVDKSRWQQGNVFSCSVMHEALHNHYTQKSLSLSPGK

SEQ ID NO: 275 - protein, 453 aa, Artificial Sequence
  PR004335|pHBM005441|HC
EVQLVESGGGLVQPGGSLRLSCAASGFTFNTYAMNWVRQAPGKGLEWVSRIRSKSNNYATYYADSVKDRFTISRDDSKSTLYLQMNSLRAEDTAVYYCVRGKENGNYYAMDYWGQGTTVTVSSASTKGPSVFPLAPSSKSTSGGTAALGCLVKDYFPEPVTVSWNSGALTSGVHTFPAVLQSSGLYSLSSVVTVPSSSLGTQTYICNVNHKPSNTKVDKKVEPKSCDKTHTCPPCPAPELLGGPDVFLFPPKPKDTLMISRTPEVTCVVVDVSHEDPEVKFNWYVDGVEVHNAKTKPREEQYNSTYRVVSVLTVLHQDWLNGKEYKCKVSNKALPAPEEKTISKAKGQPREPQVYTLPPSREEMTKNQVSLTCLVKGFYPSDIAVEWESNGQPENNYKTTPPVLDSDGSFFLYSKLTVDKSRWQQGNVFSCSVMHEALHNHYTQKSLSLSPGK

SEQ ID NO: 276 - protein, 453 aa, Artificial Sequence
  PR004336|pHBM005443|HC; PR004521|pHBM005443|HC; PR004524|pHBM005443|HC; PR004527|pHBM005443|HC
EVQLVESGGGLVQPGGSLKLSCAASGFTFNTYAMNWVRQASGKGLEWVGRIRSKSNNYATYYADSVKDRFTISRDDSKSTLYLQMNSLKTEDTAVYYCVRGKENGNYYAMDFWGQGTTVTVSSASTKGPSVFPLAPSSKSTSGGTAALGCLVKDYFPEPVTVSWNSGALTSGVHTFPAVLQSSGLYSLSSVVTVPSSSLGTQTYICNVNHKPSNTKVDKKVEPKSCDKTHTCPPCPAPELLGGPDVFLFPPKPKDTLMISRTPEVTCVVVDVSHEDPEVKFNWYVDGVEVHNAKTKPREEQYNSTYRVVSVLTVLHQDWLNGKEYKCKVSNKALPAPEEKTISKAKGQPREPQVYTLPPSREEMTKNQVSLTCLVKGFYPSDIAVEWESNGQPENNYKTTPPVLDSDGSFFLYSKLTVDKSRWQQGNVFSCSVMHEALHNHYTQKSLSLSPGK

SEQ ID NO: 277 - protein, 453 aa, Artificial Sequence
  PR004337|pHBM005444|HC
EVQLVESGGGLVQPGGSLKLSCAASGFTFNTNAMNWVRQASGKGLEWVGRIRSKSNNYATYYADSVKDRFTISRDDSKSTLYLQMNSLKTEDTAVYYCVRGKENGNYYAMDFWGQGTTVTVSSASTKGPSVFPLAPSSKSTSGGTAALGCLVKDYFPEPVTVSWNSGALTSGVHTFPAVLQSSGLYSLSSVVTVPSSSLGTQTYICNVNHKPSNTKVDKKVEPKSCDKTHTCPPCPAPELLGGPDVFLFPPKPKDTLMISRTPEVTCVVVDVSHEDPEVKFNWYVDGVEVHNAKTKPREEQYNSTYRVVSVLTVLHQDWLNGKEYKCKVSNKALPAPEEKTISKAKGQPREPQVYTLPPSREEMTKNQVSLTCLVKGFYPSDIAVEWESNGQPENNYKTTPPVLDSDGSFFLYSKLTVDKSRWQQGNVFSCSVMHEALHNHYTQKSLSLSPGK

SEQ ID NO: 278 - protein, 453 aa, Artificial Sequence
  PR004338|pHBM005445|HC
EVQLVESGGGLVQPGGSLKLSCAASGFTFNTYAMNWVRQASGKGLEWVGRIRSKSNNYATYYADSVKDRFTISRDDSKSTLYLQMNSLKTEDTAVYYCVRGKENGNYYAMDYWGQGTTVTVSSASTKGPSVFPLAPSSKSTSGGTAALGCLVKDYFPEPVTVSWNSGALTSGVHTFPAVLQSSGLYSLSSVVTVPSSSLGTQTYICNVNHKPSNTKVDKKVEPKSCDKTHTCPPCPAPELLGGPDVFLFPPKPKDTLMISRTPEVTCVVVDVSHEDPEVKFNWYVDGVEVHNAKTKPREEQYNSTYRVVSVLTVLHQDWLNGKEYKCKVSNKALPAPEEKTISKAKGQPREPQVYTLPPSREEMTKNQVSLTCLVKGFYPSDIAVEWESNGQPENNYKTTPPVLDSDGSFFLYSKLTVDKSRWQQGNVFSCSVMHEALHNHYTQKSLSLSPGK

SEQ ID NO: 279 - protein, 453 aa, Artificial Sequence
  PR004660|pHBM005788|HC; PR004662|pHBM005788|HC
EVQLVESGGGLVQPGGSLRLSCAASGFTFSTYAMNWVRQAPGKGLEWVSRIRSKSNNYATYYADSVKDRFTISRDDSKSTLYLQMNSLRAEDTAVYYCVRGKENANYYAMDFWGQGTTVTVSSASTKGPSVFPLAPSSKSTSGGTAALGCLVKDYFPEPVTVSWNSGALTSGVHTFPAVLQSSGLYSLSSVVTVPSSSLGTQTYICNVNHKPSNTKVDKKVEPKSCDKTHTCPPCPAPELLGGPDVFLFPPKPKDTLMISRTPEVTCVVVDVSHEDPEVKFNWYVDGVEVHNAKTKPREEQYNSTYRVVSVLTVLHQDWLNGKEYKCKVSNKALPAPEEKTISKAKGQPREPQVYTLPPSREEMTKNQVSLTCLVKGFYPSDIAVEWESNGQPENNYKTTPPVLDSDGSFFLYSKLTVDKSRWQQGNVFSCSVMHEALHNHYTQKSLSLSPGK

SEQ ID NO: 280 - protein, 453 aa, Artificial Sequence
  PR004661|pHBM005789|HC; PR004663|pHBM005789|HC
EVQLVESGGGLVQPGGSLRLSCAASGFTFSTYAMNWVRQAPGKGLEWVSRIRSKSNNYATYYADSVKDRFTISRDDSKSTLYLQMNSLRAEDTAVYYCVRGKEQGNYYAMDFWGQGTTVTVSSASTKGPSVFPLAPSSKSTSGGTAALGCLVKDYFPEPVTVSWNSGALTSGVHTFPAVLQSSGLYSLSSVVTVPSSSLGTQTYICNVNHKPSNTKVDKKVEPKSCDKTHTCPPCPAPELLGGPDVFLFPPKPKDTLMISRTPEVTCVVVDVSHEDPEVKFNWYVDGVEVHNAKTKPREEQYNSTYRVVSVLTVLHQDWLNGKEYKCKVSNKALPAPEEKTISKAKGQPREPQVYTLPPSREEMTKNQVSLTCLVKGFYPSDIAVEWESNGQPENNYKTTPPVLDSDGSFFLYSKLTVDKSRWQQGNVFSCSVMHEALHNHYTQKSLSLSPGK

SEQ ID NO: 281 - protein, 453 aa, Artificial Sequence
  PR004664|pHBM005786|HC; PR004666|pHBM005786|HC
EVQLVESGGGLVKPGGSLRLSCAASGFTFSTYAMNWVRQAPGKGLEWVGRIRSKSNNYATYYADSVKDRFTISRDDSKSTLYLQMNSLKTEDTAVYYCVRGKENANYYAMDFWGQGTTVTVSSASTKGPSVFPLAPSSKSTSGGTAALGCLVKDYFPEPVTVSWNSGALTSGVHTFPAVLQSSGLYSLSSVVTVPSSSLGTQTYICNVNHKPSNTKVDKKVEPKSCDKTHTCPPCPAPELLGGPDVFLFPPKPKDTLMISRTPEVTCVVVDVSHEDPEVKFNWYVDGVEVHNAKTKPREEQYNSTYRVVSVLTVLHQDWLNGKEYKCKVSNKALPAPEEKTISKAKGQPREPQVYTLPPSREEMTKNQVSLTCLVKGFYPSDIAVEWESNGQPENNYKTTPPVLDSDGSFFLYSKLTVDKSRWQQGNVFSCSVMHEALHNHYTQKSLSLSPGK

SEQ ID NO: 282 - protein, 453 aa, Artificial Sequence
  PR004665|pHBM005787|HC; PR004667|pHBM005787|HC
EVQLVESGGGLVKPGGSLRLSCAASGFTFSTYAMNWVRQAPGKGLEWVGRIRSKSNNYATYYADSVKDRFTISRDDSKSTLYLQMNSLKTEDTAVYYCVRGKEQGNYYAMDFWGQGTTVTVSSASTKGPSVFPLAPSSKSTSGGTAALGCLVKDYFPEPVTVSWNSGALTSGVHTFPAVLQSSGLYSLSSVVTVPSSSLGTQTYICNVNHKPSNTKVDKKVEPKSCDKTHTCPPCPAPELLGGPDVFLFPPKPKDTLMISRTPEVTCVVVDVSHEDPEVKFNWYVDGVEVHNAKTKPREEQYNSTYRVVSVLTVLHQDWLNGKEYKCKVSNKALPAPEEKTISKAKGQPREPQVYTLPPSREEMTKNQVSLTCLVKGFYPSDIAVEWESNGQPENNYKTTPPVLDSDGSFFLYSKLTVDKSRWQQGNVFSCSVMHEALHNHYTQKSLSLSPGK

SEQ ID NO: 283 - protein, 453 aa, Artificial Sequence
  PR004668|pHBM005792|HC
EVQLVESGGGLVQPGGSLRLSCAASGFTFNTYAMNWVRQAPGKGLEWVSRIRSKSNNYATYYADSVKDRFTISRDDSKSTLYLQMNSLRAEDTAVYYCVRGKENGNYYAMDFWGQGTTVTVSSASTKGPSVFPLAPSSKSTSGGTAALGCLVKDYFPEPVTVSWNSGALTSGVHTFPAVLQSSGLYSLSSVVTVPSSSLGTQTYICNVNHKPSNTKVDKKVEPKSCDKTHTCPPCPAPELLGGPSVFLFPPKPKDTLMISRTPEVTCVVVDVSHEDPEVKFNWYVDGVEVHNAKTKPREEQYNSTYRVVSVLTVLHQDWLNGKEYKCKVSNKALPAPIEKTISKAKGQPREPQVYTLPPSREEMTKNQVSLTCLVKGFYPSDIAVEWESNGQPENNYKTTPPVLDSDGSFFLYSKLTVDKSRWQQGNVFSCSVMHEALHNHYTQKSLSLSPGK

SEQ ID NO: 284 - protein, 453 aa, Artificial Sequence
  PR004669|pHBM005793|HC
EVQLVESGGGLVKPGGSLRLSCAASGFTFNTYAMNWVRQAPGKGLEWVGRIRSKSNNYATYYADSVKDRFTISRDDSKSTLYLQMNSLKTEDTAVYYCVRGKENGNYYAMDFWGQGTTVTVSSASTKGPSVFPLAPSSKSTSGGTAALGCLVKDYFPEPVTVSWNSGALTSGVHTFPAVLQSSGLYSLSSVVTVPSSSLGTQTYICNVNHKPSNTKVDKKVEPKSCDKTHTCPPCPAPELLGGPSVFLFPPKPKDTLMISRTPEVTCVVVDVSHEDPEVKFNWYVDGVEVHNAKTKPREEQYNSTYRVVSVLTVLHQDWLNGKEYKCKVSNKALPAPIEKTISKAKGQPREPQVYTLPPSREEMTKNQVSLTCLVKGFYPSDIAVEWESNGQPENNYKTTPPVLDSDGSFFLYSKLTVDKSRWQQGNVFSCSVMHEALHNHYTQKSLSLSPGK

SEQ ID NO: 285 - protein, 445 aa, Artificial Sequence
  PR004970|pHBM006115|HC
EVQLVESGGGLVQPGGSLRLSCAASGFTFSSYWMSWVPQAPGKGLEWVANIKQDGSAKFYVDSVKGRFTISRDNAKNSLYLQMNSLRAEDTAVYYCARSWGFAYWGQGTLVTVSSASTKGPSVFPLAPSSKSTSGGTAALGCLVKDYFPEPVTVSWNSGALTSGVHTFPAVLQSSGLYSLSSVVTVPSSSLGTQTYICNVNHKPSNTKVDKKVEPKSCDKTHTCPPCPAPELLGGPSVFLFPPKPKDTLMISRTPEVTCVVVDVSHEDPEVKFNWYVDGVEVHNAKTKPREEQYNSTYRVVSVLTVLHQDWLNGKEYKCKVSNKALPAPIEKTISKAKGQPREPQVYTLPPSREEMTKNQVSLTCLVKGFYPSDIAVEWESNGQPENNYKTTPPVLDSDGSFFLYSKLTVDKSRWQQGNVFSCSVMHEALHNHYTQKSLSLSPGK

SEQ ID NO: 286 - protein, 457 aa, Artificial Sequence
  PR004974|pHBM006117|HC
QITLKESGPTLVKPTQTLTLTCTFSGFSLSTSGVGVGWIRQPPGKALEWLALIYWNDDKRYSPSLKSRLTITKDTSKNQVVLTMTNMDPVDTATYYCAHRRLRYSGRYYYYYGTDVWGQGTTVTVSSASTKGPSVFPLAPSSKSTSGGTAALGCLVKDYFPEPVTVSWNSGALTSGVHTFPAVLQSSGLYSLSSVVTVPSSSLGTQTYICNVNHKPSNTKVDKKVEPKSCDKTHTCPPCPAPELLGGPSVFLFPPKPKDTLMISRTPEVTCVVVDVSHEDPEVKFNWYVDGVEVHNAKTKPREEQYNSTYRVVSVLTVLHQDWLNGKEYKCKVSNKALPAPIEKTISKAKGQPREPQVYTLPPSREEMTKNQVSLTCLVKGFYPSDIAVEWESNGQPENNYKTTPPVLDSDGSFFLYSKLTVDKSRWQQGNVFSCSVMHEALHNHYTQKSLSLSPGK

SEQ ID NO: 287 - protein, 452 aa, Artificial Sequence
  PR005124|pHBM006274|HC
QVQLVESGGGVVQPGRSLRLSCVASGFTFSSYGMHWVRQAPGKGLEWVAVIWHDGSNIFYADSVKGRFTISRDNSKNTLYLQMNSLRAEDTAVYWCARHRRSDYWYYGMDVWGQGTTVTVSSASTKGPSVFPLAPSSKSTSGGTAALGCLVKDYFPEPVTVSWNSGALTSGVHTFPAVLQSSGLYSLSSVVTVPSSSLGTQTYICNVNHKPSNTKVDKKVEPKSCDKTHTCPPCPAPELLGGPSVFLFPPKPKDTLMISRTPEVTCVVVDVSHEDPEVKFNWYVDGVEVHNAKTKPREEQYNSTYRVVSVLTVLHQDWLNGKEYKCKVSNKALPAPIEKTISKAKGQPREPQVYTLPPSREEMTKNQVSLTCLVKGFYPSDIAVEWESNGQPENNYKTTPPVLDSDGSFFLYSKLTVDKSRWQQGNVFSCSVMHEALHNHYTQKSLSLSPGK

SEQ ID NO: 288 - protein, 454 aa, Artificial Sequence
  PR005125|pHBM006276|HC
QVQLVESGGGVVQPGRSLRLSCAASGFTFSSYGMHWVRQVPGKGLEWVAVIWYDGSKKYYADSVKGRFTISRDNSKNTLYLQMNSLRAEDTAVYYCARGGFYYGSGNYSLFDYWGQGTLVTVSSASTKGPSVFPLAPSSKSTSGGTAALGCLVKDYFPEPVTVSWNSGALTSGVHTFPAVLQSSGLYSLSSVVTVPSSSLGTQTYICNVNHKPSNTKVDKKVEPKSCDKTHTCPPCPAPELLGGPSVFLFPPKPKDTLMISRTPEVTCVVVDVSHEDPEVKFNWYVDGVEVHNAKTKPREEQYNSTYRVVSVLTVLHQDWLNGKEYKCKVSNKALPAPIEKTISKAKGQPREPQVYTLPPSREEMTKNQVSLTCLVKGFYPSDIAVEWESNGQPENNYKTTPPVLDSDGSFFLYSKLTVDKSRWQQGNVFSCSVMHEALHNHYTQKSLSLSPGK

SEQ ID NO: 289 - protein, 452 aa, Artificial Sequence
  PR005127|pHBM006280|HC
QVQLVESGGGVVQPGRSLRLSCVASGFTFSSYGMHWVRQAPGKGLEWVAVIWHDGSNIFYADSVKGRFTISRDNSKNTLYLQMNSLRAEDTAVYWCARHRRSDYWYYGMDVWGQGTTVTVSSASTKGPSVFPLAPSSKSTSGGTAALGCLVKDYFPEPVTVSWNSGALTSGVHTFPAVLQSSGLYSLSSVVTVPSSSLGTQTYICNVNHKPSNTKVDKKVEPKSCDKTHTCPPCPAPELLGGPDVFLFPPKPKDTLMISRTPEVTCVVVDVSHEDPEVKFNWYVDGVEVHNAKTKPREEQYNSTYRVVSVLTVLHQDWLNGKEYKCKVSNKALPAPEEKTISKAKGQPREPQVYTLPPSREEMTKNQVSLTCLVKGFYPSDIAVEWESNGQPENNYKTTPPVLDSDGSFFLYSKLTVDKSRWQQGNVFSCSVMHEALHNHYTQKSLSLSPGK

SEQ ID NO: 290 - protein, 454 aa, Artificial Sequence
  PR005128|pHBM006281|HC
QVQLVESGGGVVQPGRSLRLSCAASGFTFSSYGMHWVRQVPGKGLEWVAVIWYDGSKKYYADSVKGRFTISRDNSKNTLYLQMNSLRAEDTAVYYCARGGFYYGSGNYSLFDYWGQGTLVTVSSASTKGPSVFPLAPSSKSTSGGTAALGCLVKDYFPEPVTVSWNSGALTSGVHTFPAVLQSSGLYSLSSVVTVPSSSLGTQTYICNVNHKPSNTKVDKKVEPKSCDKTHTCPPCPAPELLGGPDVFLFPPKPKDTLMISRTPEVTCVVVDVSHEDPEVKFNWYVDGVEVHNAKTKPREEQYNSTYRVVSVLTVLHQDWLNGKEYKCKVSNKALPAPEEKTISKAKGQPREPQVYTLPPSREEMTKNQVSLTCLVKGFYPSDIAVEWESNGQPENNYKTTPPVLDSDGSFFLYSKLTVDKSRWQQGNVFSCSVMHEALHNHYTQKSLSLSPGK

SEQ ID NO: 291 - protein, 457 aa, Artificial Sequence
  PR005293|pHBM006504|HC
QITLKESGPTLVKPTQTLTLTCTFSGFSLSTSGVGVGWIRQPPGKALEWLALIYWNDDKRYSPSLKSRLTITKDTSKNQVVLTMTNMDPVDTATYYCAHRRLRYSGRYYYYYGTDVWGQGTTVTVSSASTKGPSVFPLAPSSKSTSGGTAALGCLVKDYFPEPVTVSWNSGALTSGVHTFPAVLQSSGLYSLSSVVTVPSSSLGTQTYICNVNHKPSNTKVDKKVEPKSCDKTHTCPPCPAPELLGGPDVFLFPPKPKDTLMISRTPEVTCVVVDVSHEDPEVKFNWYVDGVEVHNAKTKPREEQYNSTYRVVSVLTVLHQDWLNGKEYKCKVSNKALPAPEEKTISKAKGQPREPQVYTLPPSREEMTKNQVSLTCLVKGFYPSDIAVEWESNGQPENNYKTTPPVLDSDGSFFLYSKLTVDKSRWQQGNVFSCSVMHEALHNHYTQKSLSLSPGK

SEQ ID NO: 292 - protein, 453 aa, Artificial Sequence
  PR005329|pHBM006537|HC
EVKLLESGGGLVQPKGSLKLSCAASGFTFNTYAMNWVRQAPGKGLEWVARIRTKSNNYATYYADSVKDRFTISRDDSHSMLYLQMNNLKTEDTAMYYCVRGKDNGNYYAMDFWGQGTSVTVSAASTKGPSVFPLAPSSKSTSGGTAALGCLVKDYFPEPVTVSWNSGALTSGVHTFPAVLQSSGLYSLSSVVTVPSSSLGTQTYICNVNHKPSNTKVDKKVEPKSCDKTHTCPPCPAPELLGGPSVFLFPPKPKDTLMISRTPEVTCVVVDVSHEDPEVKFNWYVDGVEVHNAKTKPREEQYNSTYRVVSVLTVLHQDWLNGKEYKCKVSNKALPAPIEKTISKAKGQPREPQVYTLPPSREEMTKNQVSLTCLVKGFYPSDIAVEWESNGQPENNYKTTPPVLDSDGSFFLYSKLTVDKSRWQQGNVFSCSVMHEALHNHYTQKSLSLSPGK

SEQ ID NO: 293 - protein, 453 aa, Artificial Sequence
  PR005330|pHBM006538|HC
EVKLVESGGGLVQPGGSRKLSCAASGFTFNTYAMNWVRQAPGKGLEWVARIRSKSNNYATYYADSVKDRFTISRDDSQSMLYLQMNNLKTEDTAMYYCVRGKDYGNYYAMDFWGQGTSVTVSSASTKGPSVFPLAPSSKSTSGGTAALGCLVKDYFPEPVTVSWNSGALTSGVHTFPAVLQSSGLYSLSSVVTVPSSSLGTQTYICNVNHKPSNTKVDKKVEPKSCDKTHTCPPCPAPELLGGPSVFLFPPKPKDTLMISRTPEVTCVVVDVSHEDPEVKFNWYVDGVEVHNAKTKPREEQYNSTYRVVSVLTVLHQDWLNGKEYKCKVSNKALPAPIEKTISKAKGQPREPQVYTLPPSREEMTKNQVSLTCLVKGFYPSDIAVEWESNGQPENNYKTTPPVLDSDGSFFLYSKLTVDKSRWQQGNVFSCSVMHEALHNHYTQKSLSLSPGK

SEQ ID NO: 294 - protein, 445 aa, Artificial Sequence
  PR005331|pHBM006539|HC
EVQLVESGGGLVQPGGSLRLSCAASGFTFSNYWLSWVRQAPGKGLEWVANIKQDGSAKYYVDSVKGRFTISRDNAKNSLYLQMNSLRAEDTAVYYCVRNWGFDYWGQGTLVTVSSASTKGPSVFPLAPSSKSTSGGTAALGCLVKDYFPEPVTVSWNSGALTSGVHTFPAVLQSSGLYSLSSVVTVPSSSLGTQTYICNVNHKPSNTKVDKKVEPKSCDKTHTCPPCPAPELLGGPSVFLFPPKPKDTLMISRTPEVTCVVVDVSHEDPEVKFNWYVDGVEVHNAKTKPREEQYNSTYRVVSVLTVLHQDWLNGKEYKCKVSNKALPAPIEKTISKAKGQPREPQVYTLPPSREEMTKNQVSLTCLVKGFYPSDIAVEWESNGQPENNYKTTPPVLDSDGSFFLYSKLTVDKSRWQQGNVFSCSVMHEALHNHYTQKSLSLSPGK

SEQ ID NO: 295 - protein, 453 aa, Artificial Sequence
  PR005332|pHBM006540|HC
EVKLLESGGGLVQPKGSLKLSCAASGFTFNTYAMNWVRQAPGKGLEWVARIRTKSNNYATYYADSVKDRFTISRDDSHSMLYLQMNNLKTEDTAMYYCVRGKDNGNYYAMDFWGQGTSVTVSAASTKGPSVFPLAPSSKSTSGGTAALGCLVKDYFPEPVTVSWNSGALTSGVHTFPAVLQSSGLYSLSSVVTVPSSSLGTQTYICNVNHKPSNTKVDKKVEPKSCDKTHTCPPCPAPELLGGPDVFLFPPKPKDTLMISRTPEVTCVVVDVSHEDPEVKFNWYVDGVEVHNAKTKPREEQYNSTYRVVSVLTVLHQDWLNGKEYKCKVSNKALPAPEEKTISKAKGQPREPQVYTLPPSREEMTKNQVSLTCLVKGFYPSDIAVEWESNGQPENNYKTTPPVLDSDGSFFLYSKLTVDKSRWQQGNVFSCSVMHEALHNHYTQKSLSLSPGK

SEQ ID NO: 296 - protein, 453 aa, Artificial Sequence
  PR005333|pHBM006541|HC
EVKLVESGGGLVQPGGSRKLSCAASGFTFNTYAMNWVRQAPGKGLEWVARIRSKSNNYATYYADSVKDRFTISRDDSQSMLYLQMNNLKTEDTAMYYCVRGKDYGNYYAMDFWGQGTSVTVSSASTKGPSVFPLAPSSKSTSGGTAALGCLVKDYFPEPVTVSWNSGALTSGVHTFPAVLQSSGLYSLSSVVTVPSSSLGTQTYICNVNHKPSNTKVDKKVEPKSCDKTHTCPPCPAPELLGGPDVFLFPPKPKDTLMISRTPEVTCVVVDVSHEDPEVKFNWYVDGVEVHNAKTKPREEQYNSTYRVVSVLTVLHQDWLNGKEYKCKVSNKALPAPEEKTISKAKGQPREPQVYTLPPSREEMTKNQVSLTCLVKGFYPSDIAVEWESNGQPENNYKTTPPVLDSDGSFFLYSKLTVDKSRWQQGNVFSCSVMHEALHNHYTQKSLSLSPGK

SEQ ID NO: 297 - protein, 445 aa, Artificial Sequence
  PR005335|pHBM006543|HC
QVQLVQSGGGLVQPGGSLRLSCTASGFTFSYYWLSWVRQAPGKGLEWVANIKQDGSTTYYVDSVKGRFTISRDNAKNSLYLQMNSLRAEDTAVYYCARNWGFDYWGQGTLVTVSSASTKGPSVFPLAPSSKSTSGGTAALGCLVKDYFPEPVTVSWNSGALTSGVHTFPAVLQSSGLYSLSSVVTVPSSSLGTQTYICNVNHKPSNTKVDKKVEPKSCDKTHTCPPCPAPELLGGPDVFLFPPKPKDTLMISRTPEVTCVVVDVSHEDPEVKFNWYVDGVEVHNAKTKPREEQYNSTYRVVSVLTVLHQDWLNGKEYKCKVSNKALPAPEEKTISKAKGQPREPQVYTLPPSREEMTKNQVSLTCLVKGFYPSDIAVEWESNGQPENNYKTTPPVLDSDGSFFLYSKLTVDKSRWQQGNVFSCSVMHEALHNHYTQKSLSLSPGK

SEQ ID NO: 298 - protein, 445 aa, Artificial Sequence
  PR005336|pHBM006544|HC
EVQLVESGGGLVQPGGSLRLSCAASGFTFSNYWLSWVRQAPGKGLEWVANIKQDGSAKYYVDSVKGRFTISRDNAKNSLYLQMNSLRAEDTAVYYCVRNWGFDYWGQGTLVTVSSASTKGPSVFPLAPSSKSTSGGTAALGCLVKDYFPEPVTVSWNSGALTSGVHTFPAVLQSSGLYSLSSVVTVPSSSLGTQTYICNVNHKPSNTKVDKKVEPKSCDKTHTCPPCPAPELLGGPDVFLFPPKPKDTLMISRTPEVTCVVVDVSHEDPEVKFNWYVDGVEVHNAKTKPREEQYNSTYRVVSVLTVLHQDWLNGKEYKCKVSNKALPAPEEKTISKAKGQPREPQVYTLPPSREEMTKNQVSLTCLVKGFYPSDIAVEWESNGQPENNYKTTPPVLDSDGSFFLYSKLTVDKSRWQQGNVFSCSVMHEALHNHYTQKSLSLSPGK

SEQ ID NO: 299 - protein, 453 aa, Artificial Sequence
  PR005565|pHBM006805|HC
EVQLVESGGGLVKPGGSLRLSCAASGFTFSTYAMNWVRQAPGKGLEWVGRIRSKSNNYATYYADSVKDRFTISRDDSKSTLYLQMNSLKTEDTAVYYCVRGKENANYYAMDFWGQGTTVTVSSASTKGPSVFPLAPSSKSTSGGTAALGCLVKDYFPEPVTVSWNSGALTSGVHTFPAVLQSSGLYSLSSVVTVPSSSLGTQTYICNVNHKPSNTKVDKKVEPKSCDKTHTCPPCPAPELLGGPSVFLFPPKPKDTLMISRTPEVTCVVVDVSHEDPEVKFNWYVDGVEVHNAKTKPREEQYNSTYRVVSVLTVLHQDWLNGKEYKCKVSNKALPAPIEKTISKAKGQPREPQVYTLPPSREEMTKNQVSLTCLVKGFYPSDIAVEWESNGQPENNYKTTPPVLDSDGSFFLYSKLTVDKSRWQQGNVFSCSVMHEALHNHYTQKSLSLSPGK

SEQ ID NO: 300 - protein, 226 aa, Artificial Sequence
  PR005750|pHBM007021|HC
EVQLVESGGGLVKPGGSLRLSCAASGFTFSTYAMNWVRQAPGKGLEWVGRIRSKSNNYATYYADSVKDRFTISRDDSKSTLYLQMNSLKTEDTAVYYCVRGKENANYYAMDFWGQGTTVTVSSASTKGPSVFPLAPSSKSTSGGTAALGCLVKDYFPEPVTVSWNSGALTSGVHTFPAVLQSSGLYSLSSVVTVPSSSLGTQTYICNVNHKPSNTKVDKKVEPKSC

SEQ ID NO: 301 - protein, 226 aa, Artificial Sequence
  PR005751|pHBM007019|HC
EVQLVESGGGLVKPGGSLRLSCAASGFTFSTYAMNWVRQAPGKGLEWVGRIRSKSNNYATYYADSVKDRFTISRDDSKSTLYLQMNSLKTEDTAVYYCVRGKEHGNYYAMDFWGQGTTVTVSSASTKGPSVFPLAPSSKSTSGGTAALGCLVKDYFPEPVTVSWNSGALTSGVHTFPAVLQSSGLYSLSSVVTVPSSSLGTQTYICNVNHKPSNTKVDKKVEPKSC

SEQ ID NO: 302 - protein, 226 aa, Artificial Sequence
  PR005752|pHBM007009|HC
EVQLVESGGGLVKPGGSLRLSCAASGFTFSTYAMNWVRQAPGKGLEWVGRIRSKSNYYATYYADSVKDRFTISRDDSKSTLYLQMNSLKTEDTAVYYCVRGKEHGNYYAMDFWGQGTTVTVSSASTKGPSVFPLAPSSKSTSGGTAALGCLVKDYFPEPVTVSWNSGALTSGVHTFPAVLQSSGLYSLSSVVTVPSSSLGTQTYICNVNHKPSNTKVDKKVEPKSC

SEQ ID NO: 303 - protein, 226 aa, Artificial Sequence
  PR005753|pHBM007020|HC
EVQLVESGGGLVKPGGSLRLSCAASGFTFSTYAMNWVRQAPGKGLEWVGRIRSKSNNYATYYADSVKDRFTISRDDSKSTLYLQMNSLKTEDTAVYYCVRGKEIGNYYAMDFWGQGTTVTVSSASTKGPSVFPLAPSSKSTSGGTAALGCLVKDYFPEPVTVSWNSGALTSGVHTFPAVLQSSGLYSLSSVVTVPSSSLGTQTYICNVNHKPSNTKVDKKVEPKSC

SEQ ID NO: 304 - protein, 226 aa, Artificial Sequence
  PR005754|pHBM007010|HC
EVQLVESGGGLVKPGGSLRLSCAASGFTFSTYAMNWVRQAPGKGLEWVGRIRSKSNYYATYYADSVKDRFTISRDDSKSTLYLQMNSLKTEDTAVYYCVRGKEIGNYYAMDFWGQGTTVTVSSASTKGPSVFPLAPSSKSTSGGTAALGCLVKDYFPEPVTVSWNSGALTSGVHTFPAVLQSSGLYSLSSVVTVPSSSLGTQTYICNVNHKPSNTKVDKKVEPKSC

SEQ ID NO: 305 - protein, 226 aa, Artificial Sequence
  PR005763|pHBM007005|HC
EVQLVESGGGLVKPGGSLRLSCAASGFTFSTYAMNWVRQAPGKGLEWVGRIRSKSNYYATYYADSVKDRFTISRDDSKSTLYLQMNSLKTEDTAVYYCVRGKEHGKYYAMDFWGQGTTVTVSSASTKGPSVFPLAPSSKSTSGGTAALGCLVKDYFPEPVTVSWNSGALTSGVHTFPAVLQSSGLYSLSSVVTVPSSSLGTQTYICNVNHKPSNTKVDKKVEPKSC

SEQ ID NO: 306 - protein, 226 aa, Artificial Sequence
  PR005787|pHBM007006|HC
EVQLVESGGGLVKPGGSLRLSCAASGFTFSTYAMNWVRQAPGKGLEWVGRIRSKSNYYATYYADSVKDRFTISRDDSKSTLYLQMNSLKTEDTAVYYCVRGKEIGKYYAMDFWGQGTTVTVSSASTKGPSVFPLAPSSKSTSGGTAALGCLVKDYFPEPVTVSWNSGALTSGVHTFPAVLQSSGLYSLSSVVTVPSSSLGTQTYICNVNHKPSNTKVDKKVEPKSC

SEQ ID NO: 307 - protein, 453 aa, Artificial Sequence
  PR006154|pHBM007001|HC
EVQLVESGGGLVKPGGSLRLSCAASGFTFSTYAMNWVRQAPGKGLEWVGRIRSKSNNYATYYADSVKDRFTISRDDSKSTLYLQMNSLKTEDTAVYYCVRGKEHGNYYAMDFWGQGTTVTVSSASTKGPSVFPLAPSSKSTSGGTAALGCLVKDYFPEPVTVSWNSGALTSGVHTFPAVLQSSGLYSLSSVVTVPSSSLGTQTYICNVNHKPSNTKVDKKVEPKSCDKTHTCPPCPAPELLGGPDVFLFPPKPKDTLMISRTPEVTCVVVDVSHEDPEVKFNWYVDGVEVHNAKTKPREEQYNSTYRVVSVLTVLHQDWLNGKEYKCKVSNKALPAPEEKTISKAKGQPREPQVYTLPPSREEMTKNQVSLTCLVKGFYPSDIAVEWESNGQPENNYKTTPPVLDSDGSFFLYSKLTVDKSRWQQGNVFSCSVMHEALHNHYTQKSLSLSPGK

SEQ ID NO: 308 - protein, 453 aa, Artificial Sequence
  PR006155|pHBM006991|HC
EVQLVESGGGLVKPGGSLRLSCAASGFTFSTYAMNWVRQAPGKGLEWVGRIRSKSNYYATYYADSVKDRFTISRDDSKSTLYLQMNSLKTEDTAVYYCVRGKEHGNYYAMDFWGQGTTVTVSSASTKGPSVFPLAPSSKSTSGGTAALGCLVKDYFPEPVTVSWNSGALTSGVHTFPAVLQSSGLYSLSSVVTVPSSSLGTQTYICNVNHKPSNTKVDKKVEPKSCDKTHTCPPCPAPELLGGPDVFLFPPKPKDTLMISRTPEVTCVVVDVSHEDPEVKFNWYVDGVEVHNAKTKPREEQYNSTYRVVSVLTVLHQDWLNGKEYKCKVSNKALPAPEEKTISKAKGQPREPQVYTLPPSREEMTKNQVSLTCLVKGFYPSDIAVEWESNGQPENNYKTTPPVLDSDGSFFLYSKLTVDKSRWQQGNVFSCSVMHEALHNHYTQKSLSLSPGK

SEQ ID NO: 309 - protein, 453 aa, Artificial Sequence
  PR006156|pHBM007002|HC
EVQLVESGGGLVKPGGSLRLSCAASGFTFSTYAMNWVRQAPGKGLEWVGRIRSKSNNYATYYADSVKDRFTISRDDSKSTLYLQMNSLKTEDTAVYYCVRGKEIGNYYAMDFWGQGTTVTVSSASTKGPSVFPLAPSSKSTSGGTAALGCLVKDYFPEPVTVSWNSGALTSGVHTFPAVLQSSGLYSLSSVVTVPSSSLGTQTYICNVNHKPSNTKVDKKVEPKSCDKTHTCPPCPAPELLGGPDVFLFPPKPKDTLMISRTPEVTCVVVDVSHEDPEVKFNWYVDGVEVHNAKTKPREEQYNSTYRVVSVLTVLHQDWLNGKEYKCKVSNKALPAPEEKTISKAKGQPREPQVYTLPPSREEMTKNQVSLTCLVKGFYPSDIAVEWESNGQPENNYKTTPPVLDSDGSFFLYSKLTVDKSRWQQGNVFSCSVMHEALHNHYTQKSLSLSPGK

SEQ ID NO: 310 - protein, 453 aa, Artificial Sequence
  PR006157|pHBM006992|HC
EVQLVESGGGLVKPGGSLRLSCAASGFTFSTYAMNWVRQAPGKGLEWVGRIRSKSNYYATYYADSVKDRFTISRDDSKSTLYLQMNSLKTEDTAVYYCVRGKEIGNYYAMDFWGQGTTVTVSSASTKGPSVFPLAPSSKSTSGGTAALGCLVKDYFPEPVTVSWNSGALTSGVHTFPAVLQSSGLYSLSSVVTVPSSSLGTQTYICNVNHKPSNTKVDKKVEPKSCDKTHTCPPCPAPELLGGPDVFLFPPKPKDTLMISRTPEVTCVVVDVSHEDPEVKFNWYVDGVEVHNAKTKPREEQYNSTYRVVSVLTVLHQDWLNGKEYKCKVSNKALPAPEEKTISKAKGQPREPQVYTLPPSREEMTKNQVSLTCLVKGFYPSDIAVEWESNGQPENNYKTTPPVLDSDGSFFLYSKLTVDKSRWQQGNVFSCSVMHEALHNHYTQKSLSLSPGK

SEQ ID NO: 311 - protein, 453 aa, Artificial Sequence
  PR006161|pHBM006987|HC
EVQLVESGGGLVKPGGSLRLSCAASGFTFSTYAMNWVRQAPGKGLEWVGRIRSKSNYYATYYADSVKDRFTISRDDSKSTLYLQMNSLKTEDTAVYYCVRGKEHGKYYAMDFWGQGTTVTVSSASTKGPSVFPLAPSSKSTSGGTAALGCLVKDYFPEPVTVSWNSGALTSGVHTFPAVLQSSGLYSLSSVVTVPSSSLGTQTYICNVNHKPSNTKVDKKVEPKSCDKTHTCPPCPAPELLGGPDVFLFPPKPKDTLMISRTPEVTCVVVDVSHEDPEVKFNWYVDGVEVHNAKTKPREEQYNSTYRVVSVLTVLHQDWLNGKEYKCKVSNKALPAPEEKTISKAKGQPREPQVYTLPPSREEMTKNQVSLTCLVKGFYPSDIAVEWESNGQPENNYKTTPPVLDSDGSFFLYSKLTVDKSRWQQGNVFSCSVMHEALHNHYTQKSLSLSPGK

SEQ ID NO: 312 - protein, 453 aa, Artificial Sequence
  PR006166|pHBM006988|HC
EVQLVESGGGLVKPGGSLRLSCAASGFTFSTYAMNWVRQAPGKGLEWVGRIRSKSNYYATYYADSVKDRFTISRDDSKSTLYLQMNSLKTEDTAVYYCVRGKEIGKYYAMDFWGQGTTVTVSSASTKGPSVFPLAPSSKSTSGGTAALGCLVKDYFPEPVTVSWNSGALTSGVHTFPAVLQSSGLYSLSSVVTVPSSSLGTQTYICNVNHKPSNTKVDKKVEPKSCDKTHTCPPCPAPELLGGPDVFLFPPKPKDTLMISRTPEVTCVVVDVSHEDPEVKFNWYVDGVEVHNAKTKPREEQYNSTYRVVSVLTVLHQDWLNGKEYKCKVSNKALPAPEEKTISKAKGQPREPQVYTLPPSREEMTKNQVSLTCLVKGFYPSDIAVEWESNGQPENNYKTTPPVLDSDGSFFLYSKLTVDKSRWQQGNVFSCSVMHEALHNHYTQKSLSLSPGK

SEQ ID NO: 313 - protein, 453 aa, Artificial Sequence
  PR006272|pHBM007521|HC
EVQLVESGGGLVKPGGSLRLSCAASGFTFSTYAMNWVRQAPGKGLEWVGRIRSKSNNYATYYADSVKDRFTISRDDSKSTLYLQMNSLKTEDTAVYYCVRGKEHGNYYAMDFWGQGTTVTVSSASTKGPSVFPLAPSSKSTSGGTAALGCLVKDYFPEPVTVSWNSGALTSGVHTFPAVLQSSGLYSLSSVVTVPSSSLGTQTYICNVNHKPSNTKVDKKVEPKSCDKTHTCPPCPAPELLGGPSVFLFPPKPKDTLMISRTPEVTCVVVDVSHEDPEVKFNWYVDGVEVHNAKTKPREEQYNSTYRVVSVLTVLHQDWLNGKEYKCKVSNKALPAPIEKTISKAKGQPREPQVYTLPPSREEMTKNQVSLTCLVKGFYPSDIAVEWESNGQPENNYKTTPPVLDSDGSFFLYSKLTVDKSRWQQGNVFSCSVMHEALHNHYTQKSLSLSPGK

SEQ ID NO: 314 - protein, 453 aa, Artificial Sequence
  PR006273|pHBM007522|HC
EVQLVESGGGLVKPGGSLRLSCAASGFTFSTYAMNWVRQAPGKGLEWVGRIRSKSNNYATYYADSVKDRFTISRDDSKSTLYLQMNSLKTEDTAVYYCVRGKEIGNYYAMDFWGQGTTVTVSSASTKGPSVFPLAPSSKSTSGGTAALGCLVKDYFPEPVTVSWNSGALTSGVHTFPAVLQSSGLYSLSSVVTVPSSSLGTQTYICNVNHKPSNTKVDKKVEPKSCDKTHTCPPCPAPELLGGPSVFLFPPKPKDTLMISRTPEVTCVVVDVSHEDPEVKFNWYVDGVEVHNAKTKPREEQYNSTYRVVSVLTVLHQDWLNGKEYKCKVSNKALPAPIEKTISKAKGQPREPQVYTLPPSREEMTKNQVSLTCLVKGFYPSDIAVEWESNGQPENNYKTTPPVLDSDGSFFLYSKLTVDKSRWQQGNVFSCSVMHEALHNHYTQKSLSLSPGK

SEQ ID NO: 315 - protein, 453 aa, Artificial Sequence
  PR006274|pHBM007523|HC
EVQLVESGGGLVKPGGSLRLSCAASGFTFSTYAMNWVRQAPGKGLEWVGRIRSKSNYYATYYADSVKDRFTISRDDSKSTLYLQMNSLKTEDTAVYYCVRGKEHGKYYAMDFWGQGTTVTVSSASTKGPSVFPLAPSSKSTSGGTAALGCLVKDYFPEPVTVSWNSGALTSGVHTFPAVLQSSGLYSLSSVVTVPSSSLGTQTYICNVNHKPSNTKVDKKVEPKSCDKTHTCPPCPAPELLGGPSVFLFPPKPKDTLMISRTPEVTCVVVDVSHEDPEVKFNWYVDGVEVHNAKTKPREEQYNSTYRVVSVLTVLHQDWLNGKEYKCKVSNKALPAPIEKTISKAKGQPREPQVYTLPPSREEMTKNQVSLTCLVKGFYPSDIAVEWESNGQPENNYKTTPPVLDSDGSFFLYSKLTVDKSRWQQGNVFSCSVMHEALHNHYTQKSLSLSPGK

SEQ ID NO: 316 - protein, 453 aa, Artificial Sequence
  PR006275|pHBM007524|HC
EVQLVESGGGLVKPGGSLRLSCAASGFTFSTYAMNWVRQAPGKGLEWVGRIRSKSNYYATYYADSVKDRFTISRDDSKSTLYLQMNSLKTEDTAVYYCVRGKEIGKYYAMDFWGQGTTVTVSSASTKGPSVFPLAPSSKSTSGGTAALGCLVKDYFPEPVTVSWNSGALTSGVHTFPAVLQSSGLYSLSSVVTVPSSSLGTQTYICNVNHKPSNTKVDKKVEPKSCDKTHTCPPCPAPELLGGPSVFLFPPKPKDTLMISRTPEVTCVVVDVSHEDPEVKFNWYVDGVEVHNAKTKPREEQYNSTYRVVSVLTVLHQDWLNGKEYKCKVSNKALPAPIEKTISKAKGQPREPQVYTLPPSREEMTKNQVSLTCLVKGFYPSDIAVEWESNGQPENNYKTTPPVLDSDGSFFLYSKLTVDKSRWQQGNVFSCSVMHEALHNHYTQKSLSLSPGK

SEQ ID NO: 317 - protein, 453 aa, Artificial Sequence
  PR006276|pHBM007525|HC
EVQLVESGGGLVKPGGSLRLSCAASGFTFSTYAMNWVRQAPGKGLEWVGRIRSKSNYYATYYADSVKDRFTISRDDSKSTLYLQMNSLKTEDTAVYYCVRGKEHGNYYAMDFWGQGTTVTVSSASTKGPSVFPLAPSSKSTSGGTAALGCLVKDYFPEPVTVSWNSGALTSGVHTFPAVLQSSGLYSLSSVVTVPSSSLGTQTYICNVNHKPSNTKVDKKVEPKSCDKTHTCPPCPAPELLGGPSVFLFPPKPKDTLMISRTPEVTCVVVDVSHEDPEVKFNWYVDGVEVHNAKTKPREEQYNSTYRVVSVLTVLHQDWLNGKEYKCKVSNKALPAPIEKTISKAKGQPREPQVYTLPPSREEMTKNQVSLTCLVKGFYPSDIAVEWESNGQPENNYKTTPPVLDSDGSFFLYSKLTVDKSRWQQGNVFSCSVMHEALHNHYTQKSLSLSPGK

SEQ ID NO: 318 - protein, 453 aa, Artificial Sequence
  PR006277|pHBM007526|HC
EVQLVESGGGLVKPGGSLRLSCAASGFTFSTYAMNWVRQAPGKGLEWVGRIRSKSNYYATYYADSVKDRFTISRDDSKSTLYLQMNSLKTEDTAVYYCVRGKEIGNYYAMDFWGQGTTVTVSSASTKGPSVFPLAPSSKSTSGGTAALGCLVKDYFPEPVTVSWNSGALTSGVHTFPAVLQSSGLYSLSSVVTVPSSSLGTQTYICNVNHKPSNTKVDKKVEPKSCDKTHTCPPCPAPELLGGPSVFLFPPKPKDTLMISRTPEVTCVVVDVSHEDPEVKFNWYVDGVEVHNAKTKPREEQYNSTYRVVSVLTVLHQDWLNGKEYKCKVSNKALPAPIEKTISKAKGQPREPQVYTLPPSREEMTKNQVSLTCLVKGFYPSDIAVEWESNGQPENNYKTTPPVLDSDGSFFLYSKLTVDKSRWQQGNVFSCSVMHEALHNHYTQKSLSLSPGK

SEQ ID NO: 319 - protein, 219 aa, Artificial Sequence
  PR004120|pHBM005098|LC
DIVMTQAATSVLVTPGESVSISCRSSKSLLYSNGNTYLYWFLQRPGQSPQLLIYRMSNLASGVPDRFSGSGSGTAFTLRISRVEAEDVGVYYCMQHLEYPFTFGGGTKLEIKRTVAAPSVFIFPPSDEQLKSGTASVVCLLNNFYPREAKVQWKVDNALQSGNSQESVTEQDSKDSTYSLSSTLTLSKADYEKHKVYACEVTHQGLSSPVTKSFNRGEC

SEQ ID NO: 320 - protein, 219 aa, Artificial Sequence
  PR004121|pHBM005099|LC
DIVITQAAPSVPVTPGESVSISCRSSKSLLHSNGNTYLYWFLQRPGQSPQLLIYRMSNLASGVPDRFSGSGSGTAFTLRISRVEAEDVGVYYCMQHLEYPFTFGGGTKLEMKRTVAAPSVFIFPPSDEQLKSGTASVVCLLNNFYPREAKVQWKVDNALQSGNSQESVTEQDSKDSTYSLSSTLTLSKADYEKHKVYACEVTHQGLSSPVTKSFNRGEC

SEQ ID NO: 321 - protein, 219 aa, Artificial Sequence
  PR004122|pHBM005100|LC; PR004249|pHBM005100|LC
DIVMTQAAPSVPVTPGESVSISCRSSKSLLHSNGNTYLYWFLQRPGQSPQLLIYRMSNLASGVPDRFSGSGSGTAFTLRISRVEAEDVGVYYCMQHLEYPLTFGAGTKLELKRTVAAPSVFIFPPSDEQLKSGTASVVCLLNNFYPREAKVQWKVDNALQSGNSQESVTEQDSKDSTYSLSSTLTLSKADYEKHKVYACEVTHQGLSSPVTKSFNRGEC

SEQ ID NO: 322 - protein, 219 aa, Artificial Sequence
  PR004123|pHBM005101|LC
DIVMTQAAPSVPVTPGESVSISCRSSKSLLHSNGNTYLYWFLQRPGQSPQLLIYRMSNLASGVPDRFSGSGSGTAFTLRISRVEAEDVGVYYCMQHLEYPFTFGGGTKLELKRTVAAPSVFIFPPSDEQLKSGTASVVCLLNNFYPREAKVQWKVDNALQSGNSQESVTEQDSKDSTYSLSSTLTLSKADYEKHKVYACEVTHQGLSSPVTKSFNRGEC

SEQ ID NO: 323 - protein, 219 aa, Artificial Sequence
  PR004124|pHBM005102|LC
DIVMTQDELSNPVTSGESVSISCRSSKSLLHSNGNTYLYWFLQRPGQSPQLLIYRMSNLASGVPDRFSGSGSGTAFTLRISRVEAEDVGVYYCMQHLEYPFTFGGGTKLELKRTVAAPSVFIFPPSDEQLKSGTASVVCLLNNFYPREAKVQWKVDNALQSGNSQESVTEQDSKDSTYSLSSTLTLSKADYEKHKVYACEVTHQGLSSPVTKSFNRGEC

SEQ ID NO: 324 - protein, 219 aa, Artificial Sequence
  PR004125|pHBM005103|LC; PR004250|pHBM005103|LC
DIVMTQAAPSVPVTPGESVSISCRSSKSLLHSNGNTYLYWFLQRPGQSPQLLIYRMSNLASGVPDRFSGSGSGTAFTLRISRVEAEDVGVYYCMQHLEYPLTFGAGTKLEMKRTVAAPSVFIFPPSDEQLKSGTASVVCLLNNFYPREAKVQWKVDNALQSGNSQESVTEQDSKDSTYSLSSTLTLSKADYEKHKVYACEVTHQGLSSPVTKSFNRGEC

SEQ ID NO: 325 - protein, 219 aa, Artificial Sequence
  PR004126|pHBM005104|LC
DIVITQAAPSVPVTPGESVSISCRSSKSLLHSNGNTYLYWFLQRPGQSPQLLIYRMSNLASGVPDRFSGSGSGTAFTLRISRVEAEDVGVYYCMQHLEYPFTFGAGTKLELKRTVAAPSVFIFPPSDEQLKSGTASVVCLLNNFYPREAKVQWKVDNALQSGNSQESVTEQDSKDSTYSLSSTLTLSKADYEKHKVYACEVTHQGLSSPVTKSFNRGEC

SEQ ID NO: 326 - protein, 219 aa, Artificial Sequence
  PR004127|pHBM005105|LC
DIVMTQAATSVLVTPGESVSISCRSSKSLLYSNGNTYLYWFLQRPGQSPQLLIYRMSNLASGVPDRFSGSGSGTAFTLRISRVEAEDVGVYYCMQHLEYPFTFGGGTKLEMKRTVAAPSVFIFPPSDEQLKSGTASVVCLLNNFYPREAKVQWKVDNALQSGNSQESVTEQDSKDSTYSLSSTLTLSKADYEKHKVYACEVTHQGLSSPVTKSFNRGEC

SEQ ID NO: 327 - protein, 219 aa, Artificial Sequence
  PR004128|pHBM005106|LC; PR004251|pHBM005106|LC; PR004326|pHBM005106|LC; PR004327|pHBM005106|LC; PR004328|pHBM005106|LC; PR004329|pHBM005106|LC; PR004330|pHBM005106|LC; PR004331|pHBM005106|LC; PR004332|pHBM005106|LC; PR004333|pHBM005106|LC; PR004334|pHBM005106|LC; PR004335|pHBM005106|LC; PR004336|pHBM005106|LC; PR004337|pHBM005106|LC; PR004338|pHBM005106|LC
DIVMTQAAPSVPVTPGESVSISCRSSKSLLHSNGKIYLYWFLQRPGQSPQLLIYRMSNLASGVPDRFSGSGSGTAFTLRISRVEAEDVGVYYCMQHLEYPLTFGAGTKLEIKRTVAAPSVFIFPPSDEQLKSGTASVVCLLNNFYPREAKVQWKVDNALQSGNSQESVTEQDSKDSTYSLSSTLTLSKADYEKHKVYACEVTHQGLSSPVTKSFNRGEC

SEQ ID NO: 328 - protein, 219 aa, Artificial Sequence
  PR004129|pHBM005107|LC
DILLTQSPAILSVSPGERVSFSCRSSKSLLHSNGNTYLYWFLQRPGQSPQLLIYRMSNLASGVPDRFSGSGSGTAFTLRISRVEAEDVGVYYCMQHLEYPFTFGSGTKLEINRTVAAPSVFIFPPSDEQLKSGTASVVCLLNNFYPREAKVQWKVDNALQSGNSQESVTEQDSKDSTYSLSSTLTLSKADYEKHKVYACEVTHQGLSSPVTKSFNRGEC

SEQ ID NO: 329 - protein, 219 aa, Artificial Sequence
  PR004130|pHBM005108|LC
DIVMTQAAPSVPVTPGESVSISCRSSKSLLHSNGNTYLYWFLQRPGQSPQLLIYRMSNLASGVPDRFSGSGSGTAFTLRISRVEAEDVGVYYCMQHLEYPFTFGSGTKLEIKRTVAAPSVFIFPPSDEQLKSGTASVVCLLNNFYPREAKVQWKVDNALQSGNSQESVTEQDSKDSTYSLSSTLTLSKADYEKHKVYACEVTHQGLSSPVTKSFNRGEC

SEQ ID NO: 330 - protein, 219 aa, Artificial Sequence
  PR004131|pHBM005109|LC; PR004252|pHBM005109|LC
DIVMTQAAPSVPVTPGESVSISCRSNKSLLHSNGNTYLYWFLQRPGQSPQLLIYRMSNLASGVPDRFSGSGSGTAFTLRISRVEAEDVGVYYCMQHLEYPLTFGAGTKLEIKRTVAAPSVFIFPPSDEQLKSGTASVVCLLNNFYPREAKVQWKVDNALQSGNSQESVTEQDSKDSTYSLSSTLTLSKADYEKHKVYACEVTHQGLSSPVTKSFNRGEC

SEQ ID NO: 331 - protein, 220 aa, Artificial Sequence
  PR004264|pHBM005402|LC
DVVMTQSPLSLPVTLGQPASISCRSSQSLVYSDGNTYLNWFQQRPGQSPRRLIYKVSNRDSGVPDRFSGSGSGTDFTLKISRVEAEDVGVYYCMQGTHWPPITFGQGTRLEIKRTVAAPSVFIFPPSDEQLKSGTASVVCLLNNFYPREAKVQWKVDNALQSGNSQESVTEQDSKDSTYSLSSTLTLSKADYEKHKVYACEVTHQGLSSPVTKSFNRGEC

SEQ ID NO: 332 - protein, 213 aa, Artificial Sequence
  PR004265|pHBM005404|LC
DIVLIQSPAIMSASPGEKVTISCSASSSVSYMYWYQQKPGSSPKPWIYRTSNLASGVPARFSGSGSGTSYSLTISRMEAEDAATYYCQQRSSYPPTFGAGTKLELKRTVAAPSVFIFPPSDEQLKSGTASVVCLLNNFYPREAKVQWKVDNALQSGNSQESVTEQDSKDSTYSLSSTLTLSKADYEKHKVYACEVTHQGLSSPVTKSFNRGEC

SEQ ID NO: 333 - protein, 214 aa, Artificial Sequence
  PR004275|pHBM005296|LC
DIQLTQSPSTLSASVGDRVTITCRASQSISSWLAWYQQKPGKAPKLLIYKASSLESGVPSRFSGSGSGTDFTLTISSLQPEDVATYYCQKYNSAPPTFGPGTKVDIKRTVAAPSVFIFPPSDEQLKSGTASVVCLLNNFYPREAKVQWKVDNALQSGNSQESVTEQDSKDSTYSLSSTLTLSKADYEKHKVYACEVTHQGLSSPVTKSFNRGEC

SEQ ID NO: 334 - protein, 219 aa, Artificial Sequence
  PR004324|pHBM005456|LC
DIVMTQAAPSVPVTPGESVSISCRSSKSLLHSNAKIYLYWFLQRPGQSPQLLIYRMSNLASGVPDRFSGSGSGTAFTLRISRVEAEDVGVYYCMQHLEYPLTFGAGTKLEIKRTVAAPSVFIFPPSDEQLKSGTASVVCLLNNFYPREAKVQWKVDNALQSGNSQESVTEQDSKDSTYSLSSTLTLSKADYEKHKVYACEVTHQGLSSPVTKSFNRGEC

SEQ ID NO: 335 - protein, 219 aa, Artificial Sequence
  PR004325|pHBM005457|LC
DIVMTQAAPSVPVTPGESVSISCRSSKSLLHSQGKIYLYWFLQRPGQSPQLLIYRMSNLASGVPDRFSGSGSGTAFTLRISRVEAEDVGVYYCMQHLEYPLTFGAGTKLEIKRTVAAPSVFIFPPSDEQLKSGTASVVCLLNNFYPREAKVQWKVDNALQSGNSQESVTEQDSKDSTYSLSSTLTLSKADYEKHKVYACEVTHQGLSSPVTKSFNRGEC

SEQ ID NO: 336 - protein, 219 aa, Artificial Sequence
  LC
DIVMTQSPLSLPVTPGEPASISCRSSKSLLHSNGKIYLYWFLQKPGQSPQLLIYRMSNLASGVPDRFSGSGSGTDFTLKISRVEAEDVGVYYCMQHLEYPLTFGQGTKLEIKRTVAAPSVFIFPPSDEQLKSGTASVVCLLNNFYPREAKVQWKVDNALQSGNSQESVTEQDSKDSTYSLSSTLTLSKADYEKHKVYACEVTHQGLSSPVTKSFNRGEC

SEQ ID NO: 337 - protein, 219 aa, Artificial Sequence
  PR004340|pHBM005448|LC; PR004522|pHBM005448|LC; PR004523|pHBM005448|LC; PR004524|pHBM005448|LC
DIVMTQSPLSLPVTPGEPASISCRSSKSLLHSNGNTYLYWFLQKPGQSPQLLIYRMSNLASGVPDRFSGSGSGTDFTLKISRVEAEDVGVYYCMQHLEYPLTFGQGTKLEIKRTVAAPSVFIFPPSDEQLKSGTASVVCLLNNFYPREAKVQWKVDNALQSGNSQESVTEQDSKDSTYSLSSTLTLSKADYEKHKVYACEVTHQGLSSPVTKSFNRGEC

SEQ ID NO: 338 - protein, 219 aa, Artificial Sequence
  PR004342|pHBM005450|LC
DIVMTQSPLSLPVTPGEPASISCRSSKSLLHSNGNTYLYWFLQKPGQSPQLLIYRMSNLASGVPDRFSGSGSGTDFTLKISRVEAEDVGVYYCMQHLEYPFTFGQGTKLEIKRTVAAPSVFIFPPSDEQLKSGTASVVCLLNNFYPREAKVQWKVDNALQSGNSQESVTEQDSKDSTYSLSSTLTLSKADYEKHKVYACEVTHQGLSSPVTKSFNRGEC

SEQ ID NO: 339 - protein, 219 aa, Artificial Sequence
  PR004343|pHBM005452|LC; PR004525|pHBM005452|LC; PR004526|pHBM005452|LC; PR004527|pHBM005452|LC; PR004664|pHBM005452|LC; PR004665|pHBM005452|LC; PR004669|pHBM005452|LC
DIVMTQSPLSLPVTLGQPASISCRSSKSLLHSNGKIYLYWFQQRPGQSPRLLIYRMSNLASGVPDRFSGSGSGTDFTLKISRVEAEDVGVYYCMQHLEYPLTFGQGTKLEIKRTVAAPSVFIFPPSDEQLKSGTASVVCLLNNFYPREAKVQWKVDNALQSGNSQESVTEQDSKDSTYSLSSTLTLSKADYEKHKVYACEVTHQGLSSPVTKSFNRGEC

SEQ ID NO: 340 - protein, 219 aa, Artificial Sequence
  PR004344|pHBM005453|LC
DIVMTQSPLSLPVTLGQPASISCRSSKSLLHSNGNTYLYWFQQRPGQSPRLLIYRMSNLASGVPDRFSGSGSGTDFTLKISRVEAEDVGVYYCMQHLEYPLTFGQGTKLEIKRTVAAPSVFIFPPSDEQLKSGTASVVCLLNNFYPREAKVQWKVDNALQSGNSQESVTEQDSKDSTYSLSSTLTLSKADYEKHKVYACEVTHQGLSSPVTKSFNRGEC

SEQ ID NO: 341 - protein, 219 aa, Artificial Sequence
  PR004345|pHBM005454|LC
DIVMTQSPLSLPVTLGQPASISCRSNKSLLHSNGNTYLYWFQQRPGQSPRLLIYRMSNLASGVPDRFSGSGSGTDFTLKISRVEAEDVGVYYCMQHLEYPLTFGQGTKLEIKRTVAAPSVFIFPPSDEQLKSGTASVVCLLNNFYPREAKVQWKVDNALQSGNSQESVTEQDSKDSTYSLSSTLTLSKADYEKHKVYACEVTHQGLSSPVTKSFNRGEC

SEQ ID NO: 342 - protein, 219 aa, Artificial Sequence
  PR004346|pHBM005455|LC
DIVMTQSPLSLPVTLGQPASISCRSSKSLLHSNGNTYLYWFQQRPGQSPRLLIYRMSNLASGVPDRFSGSGSGTDFTLKISRVEAEDVGVYYCMQHLEYPFTFGQGTKLEIKRTVAAPSVFIFPPSDEQLKSGTASVVCLLNNFYPREAKVQWKVDNALQSGNSQESVTEQDSKDSTYSLSSTLTLSKADYEKHKVYACEVTHQGLSSPVTKSFNRGEC

SEQ ID NO: 343 - protein, 219 aa, Artificial Sequence
  PR004662|pHBM005790|LC; PR004663|pHBM005790|LC
DIVMTQSPLSLPVTPGEPASISCRSSKSLLHSNAKIYLYWFLQKPGQSPQLLIYRMSNLASGVPDRFSGSGSGTDFTLKISRVEAEDVGVYYCMQHLEYPLTFGQGTKLEIKRTVAAPSVFIFPPSDEQLKSGTASVVCLLNNFYPREAKVQWKVDNALQSGNSQESVTEQDSKDSTYSLSSTLTLSKADYEKHKVYACEVTHQGLSSPVTKSFNRGEC

SEQ ID NO: 344 - protein, 219 aa, Artificial Sequence
  LC
DIVMTQSPLSLPVTLGQPASISCRSSKSLLHSNAKIYLYWFQQRPGQSPRLLIYRMSNLASGVPDRFSGSGSGTDFTLKISRVEAEDVGVYYCMQHLEYPLTFGQGTKLEIKRTVAAPSVFIFPPSDEQLKSGTASVVCLLNNFYPREAKVQWKVDNALQSGNSQESVTEQDSKDSTYSLSSTLTLSKADYEKHKVYACEVTHQGLSSPVTKSFNRGEC

SEQ ID NO: 345 - protein, 214 aa, Artificial Sequence
  PR004970|pHBM006122|LC
DIQMTQSPSSLSASVGDRVTITCRASQGISNYLAWYQQKPGKVPKLLIYAASTLQSGVPSRFSGSGSGTDFTLTISSLQPEDVATYYCQKYNSAPWTFGQGTKVEIKRTVAAPSVFIFPPSDEQLKSGTASVVCLLNNFYPREAKVQWKVDNALQSGNSQESVTEQDSKDSTYSLSSTLTLSKADYEKHKVYACEVTHQGLSSPVTKSFNRGEC

SEQ ID NO: 346 - protein, 214 aa, Artificial Sequence
  PR004974|pHBM006126|LC; PR005293|pHBM006126|LC
EIVMTQSPATLSVSPGERATLSCRASQSVSSNLVWYQQKPGQAPRLLIYGASIRATGIPARFSGSGSGTEFTLTISSLQSEDFAVYYCQQYNNWPYTFGQGTKLEIKRTVAAPSVFIFPPSDEQLKSGTASVVCLLNNFYPREAKVQWKVDNALQSGNSQESVTEQDSKDSTYSLSSTLTLSKADYEKHKVYACEVTHQGLSSPVTKSFNRGEC

SEQ ID NO: 347 - protein, 219 aa, Artificial Sequence
  PR005124|pHBM006275|LC; PR005127|pHBM006275|LC
DVVMTQSPLSLPVTPGEPASISCRSSQSLLHSNGYNYLDWYLQKPGQSPQLLIYLGSNRASGVPDRFSGSGSGTDFTLKISRVEAEDVGVYYCMQALQTPYTFGQGTKVDIKRTVAAPSVFIFPPSDEQLKSGTASVVCLLNNFYPREAKVQWKVDNALQSGNSQESVTEQDSKDSTYSLSSTLTLSKADYEKHKVYACEVTHQGLSSPVTKSFNRGEC

SEQ ID NO: 348 - protein, 218 aa, Artificial Sequence
  PR005125|pHBM006277|LC; PR005128|pHBM006277|LC
DIVMTQSPLSLSVTLGQPASISCRSSQSLVFSNGNTYLNWFQQRPGQSPRRLIYKVSKRDSGVPDRFSGSGSGTDFTLKISRVEAEDVGVYYCMQGTHWITFGQGTRLEIKRTVAAPSVFIFPPSDEQLKSGTASVVCLLNNFYPREAKVQWKVDNALQSGNSQESVTEQDSKDSTYSLSSTLTLSKADYEKHKVYACEVTHQGLSSPVTKSFNRGEC

SEQ ID NO: 349 - protein, 219 aa, Artificial Sequence
  PR005170|pHBM006323|LC
DIVMTQAAPSVPVTPGESVSISCRSSKSLLHSNGKIYLYWFLQRPGQSPQLLIYRMSNLASGVPDRFSGSGSGTAFTLRISRVEAEDVGVYYCMQHLEYPITFGAGTKLEIKRTVAAPSVFIFPPSDEQLKSGTASVVCLLNNFYPREAKVQWKVDNALQSGNSQESVTEQDSKDSTYSLSSTLTLSKADYEKHKVYACEVTHQGLSSPVTKSFNRGEC

SEQ ID NO: 350 - protein, 219 aa, Artificial Sequence
  PR005171|pHBM006324|LC
DIVMTQAAPSVPVTPGESVSISCRSSKSLLHSNGKIYLYWFLQRPGQSPQLLIYRMSNLASGVPDRFSGSGSGTAFTLRISRVEAEDVGVYYCMQHLEYPMTFGAGTKLEIKRTVAAPSVFIFPPSDEQLKSGTASVVCLLNNFYPREAKVQWKVDNALQSGNSQESVTEQDSKDSTYSLSSTLTLSKADYEKHKVYACEVTHQGLSSPVTKSFNRGEC

SEQ ID NO: 351 - protein, 219 aa, Artificial Sequence
  PR005172|pHBM006325|LC
DIVMTQAAPSVPVTPGESVSISCRSSKSLLHSNGKIYLYWFLQRPGQSPQLLIYRMSNLASGVPDRFSGSGSGTAFTLRISRVEAEDVGVYYCMQHLEYPVTFGAGTKLEIKRTVAAPSVFIFPPSDEQLKSGTASVVCLLNNFYPREAKVQWKVDNALQSGNSQESVTEQDSKDSTYSLSSTLTLSKADYEKHKVYACEVTHQGLSSPVTKSFNRGEC

SEQ ID NO: 352 - protein, 219 aa, Artificial Sequence
  PR005329|pHBM006545|LC; PR005332|pHBM006545|LC
DIVMTQAAPSVPVTPGESVSISCRSSKSLLHSNGNTYLYWFLQRPGQSPQLLIYRMSNLASGVPDRFSSSGSGTDFTLRISRVEAEDVGVYYCMQHLEYPFTFGAGTKLEIKRTVAAPSVFIFPPSDEQLKSGTASVVCLLNNFYPREAKVQWKVDNALQSGNSQESVTEQDSKDSTYSLSSTLTLSKADYEKHKVYACEVTHQGLSSPVTKSFNRGEC

SEQ ID NO: 353 - protein, 219 aa, Artificial Sequence
  PR005330|pHBM006546|LC; PR005333|pHBM006546|LC
DIVMTQAATSVLVTPGESVSISCRSSKSLLYSNGNTYLYWFLQRPGQSPQLLIYRMSNLASGVPDRFSGSGSGTAFTLRISRVEAEDVGVYYCMQHLEYPFTFGGGTKLELKRTVAAPSVFIFPPSDEQLKSGTASVVCLLNNFYPREAKVQWKVDNALQSGNSQESVTEQDSKDSTYSLSSTLTLSKADYEKHKVYACEVTHQGLSSPVTKSFNRGEC

SEQ ID NO: 354 - protein, 219 aa, Artificial Sequence
  PR005331|pHBM006549|LC; PR005336|pHBM006549|LC
DIVMTQSPLSLPVTLGQPASISCRSSQSLVYSNGNTYLNWFQQRPGQSPRRLIYKVSNRDSGVPDRFSGSGSGTDFTLKISRVEAEDVGVYYCMQGTHWPITFGQGTRLEIKRTVAAPSVFIFPPSDEQLKSGTASVVCLLNNFYPREAKVQWKVDNALQSGNSQESVTEQDSKDSTYSLSSTLTLSKADYEKHKVYACEVTHQGLSSPVTKSFNRGEC

SEQ ID NO: 355 - protein, 219 aa, Artificial Sequence
  PR005335|pHBM006548|LC
DVVMTQSPLSLPVTLGQPASISCRSSQSLVYSNGNTYLNWFQQRPGQSPRRLIYKVSNRDSGVPDRFSGSGSGTDFTLKISRVEAEDVGVYYCMQGTHWPITFGQGTRLEIKRTVAAPSVFIFPPSDEQLKSGTASVVCLLNNFYPREAKVQWKVDNALQSGNSQESVTEQDSKDSTYSLSSTLTLSKADYEKHKVYACEVTHQGLSSPVTKSFNRGEC

SEQ ID NO: 356 - protein, 330 aa, Artificial Sequence
  human IgG1 constant region
ASTKGPSVFPLAPSSKSTSGGTAALGCLVKDYFPEPVTVSWNSGALTSGVHTFPAVLQSSGLYSLSSVVTVPSSSLGTQTYICNVNHKPSNTKVDKKVEPKSCDKTHTCPPCPAPELLGGPSVFLFPPKPKDTLMISRTPEVTCVVVDVSHEDPEVKFNWYVDGVEVHNAKTKPREEQYNSTYRVVSVLTVLHQDWLNGKEYKCKVSNKALPAPIEKTISKAKGQPREPQVYTLPPSREEMTKNQVSLTCLVKGFYPSDIAVEWESNGQPENNYKTTPPVLDSDGSFFLYSKLTVDKSRWQQGNVFSCSVMHEALHNHYTQKSLSLSPGK

SEQ ID NO: 357 - protein, 330 aa, Artificial Sequence
  human IgG1 constant region（S239D,I332E）
ASTKGPSVFPLAPSSKSTSGGTAALGCLVKDYFPEPVTVSWNSGALTSGVHTFPAVLQSSGLYSLSSVVTVPSSSLGTQTYICNVNHKPSNTKVDKKVEPKSCDKTHTCPPCPAPELLGGPDVFLFPPKPKDTLMISRTPEVTCVVVDVSHEDPEVKFNWYVDGVEVHNAKTKPREEQYNSTYRVVSVLTVLHQDWLNGKEYKCKVSNKALPAPEEKTISKAKGQPREPQVYTLPPSREEMTKNQVSLTCLVKGFYPSDIAVEWESNGQPENNYKTTPPVLDSDGSFFLYSKLTVDKSRWQQGNVFSCSVMHEALHNHYTQKSLSLSPGK

SEQ ID NO: 358 - protein, 107 aa, Artificial Sequence [sequence omitted]

SEQ ID NO: 359 - protein, 7 aa, Artificial Sequence
  general formula of HCDR1 of monkey cross-binding activity antibody
  misc_feature (5)..(5): Xaa = Asn, Gln or Ser
  misc_feature (7)..(7): Xaa = Asn or Tyr
GFTFXTX

SEQ ID NO: 360 - protein, 12 aa, Artificial Sequence
  general formula of HCDR3 of monkey cross-binding activity antibody
  misc_feature (4)..(4): Xaa = Asn or Gln
  misc_feature (5)..(5): Xaa = Ala or Gly
  misc_feature (12)..(12): Xaa = Phe or Tyr
GKEXXNYYAMDX

SEQ ID NO: 361 - protein, 16 aa, Artificial Sequence
  general formula of LCDR1 of monkey cross-binding activity antibody
  misc_feature (3)..(3): Xaa = Asn or Ser
  misc_feature (10)..(10): Xaa = Asn or Gln
  misc_feature (11)..(11): Xaa = Ala or Gly
  misc_feature (12)..(12): Xaa = Lys or Asn
  misc_feature (13)..(13): Xaa = Ile or Thr
RSXKSLLHSXXXXYLY

SEQ ID NO: 362 - protein, 9 aa, Artificial Sequence
  general formula of LCDR3 of monkey cross-binding activity antibody
  misc_feature (8)..(8): Xaa = Ile, Leu, Met or Val
MQHLEYPXT

SEQ ID NO: 363 - protein, 7 aa, Artificial Sequence
  general formula of HCDR1 of non-monkey cross-binding activity antibody
  misc_feature (1)..(1): Xaa = Glu or Gly
  misc_feature (5)..(5): Xaa = Asn or Ser
  misc_feature (7)..(7): Xaa = Asn or Tyr
XFTFXTX

SEQ ID NO: 364 - protein, 8 aa, Artificial Sequence
  general formula of HCDR2 of non-monkey cross-binding activity antibody
  misc_feature (2)..(2): Xaa = Ser or Thr
  misc_feature (4)..(4): Xaa = Met or Ser
  misc_feature (7)..(7): Xaa = Phe or Tyr
RXKXNNXA

SEQ ID NO: 365 - protein, 12 aa, Artificial Sequence
  general formula of HCDR3 of non-monkey cross-binding activity antibody
  misc_feature (3)..(3): Xaa = Asp or Glu
  misc_feature (4)..(4): Xaa = Asn or Tyr
  misc_feature (12)..(12): Xaa = Phe or Tyr
GKXXGNYYAMDX

SEQ ID NO: 366 - protein, 16 aa, Artificial Sequence
  general formula of LCDR1 of non-monkey cross-binding activity antibody
  misc_feature (8)..(8): Xaa = His or Tyr
RSSKSLLXSNGNTYLY

SEQ ID NO: 367 - protein, 8 aa, Artificial Sequence
  general formula of HCDR2 of PR4666 mutant
  misc_feature (6)..(6): Xaa = Asn or Tyr
RSKSNXYA

SEQ ID NO: 368 - protein, 12 aa, Artificial Sequence
  general formula of HCDR3 of PR4666 mutant
  misc_feature (4)..(4): Xaa = His, Ile or Asn
  misc_feature (5)..(5): Xaa = Ala or Gly
  misc_feature (6)..(6): Xaa = Lys or Asn
GKEXXXYYAMDF